European Patent Application EP 4 406 966 A1, published July 31, 2024. Title: FUSION PROTEIN DIMER COMPRISING PD-1 AND IL-21 AND USE THEREOF. Applicant: Bionsystems Inc. The sequence listing filed with the application follows.

SEQUENCE LISTING (127 sequences)

SEQ ID NO: 1 - protein, 24 aa, synthetic construct
  REGION 1..24: note = Signal Peptide 1
MQIPQAPWPVVWAVLQLGWRPGWF

SEQ ID NO: 2 - protein, 126 aa, synthetic construct
  REGION 1..126: note = hPD-1
LDSPDRPWNPPTFSPALLVVTEGDNATFTCSFSNTSESFVLNWYRMSPSNQTDKLAAFPEDRSQPGQDCRFRVTQLPNGRDFHMSVVRARRNDSGTYLCGAISLAPKAQIKESLRAELRVTERRAE

SEQ ID NO: 3 - protein, 20 aa, synthetic construct
  REGION 1..20: note = Hinge with linker 1
GGGGSGGGGSDKTHTCPPCP

SEQ ID NO: 4 - protein, 216 aa, synthetic construct
  REGION 1..216: note = Fc(29)
APELLGGPSVFLFPPKPKDTLMISRTPEVTCVVVDVSHEDPEVKFNWYVDGVEVHNAKTKPREEQYNSTYRVVSVLTVLHRDWLNGKEYKCKVSNKALPAPIEKTISKAKGQPREPQVYTLPPSRDELTKNQVSLTCLVKGFYPSDIAVEWESNGQPENNYKTTPPVLDSDGSFFLYSKLTVDKSRWQQGNVFSCSVLHEALHNHYTQKSLSLSPG

SEQ ID NO: 5 - protein, 5 aa, synthetic construct
  REGION 1..5: note = Linker 1
GGGGS

SEQ ID NO: 6 - protein, 138 aa, synthetic construct
  REGION 1..138: note = hIL-21
HKSSSQGQDRHMIRMRQLIDIVDQLKNYVNDLVPEFLPAPEDVETNCEWSAFSCFQKAQLKSANTGNNERIINVSIKKLKRKPPSTNAGRRQKHRLTCPSCDSYEKKPPKEFLERFKSLLQKMIHQHLSSRTHGSEDS

SEQ ID NO: 7 - protein, 529 aa, synthetic construct
  REGION 1..529: note = hPD-1 D-Fc(29)-hIL-21 with signal peptide
MQIPQAPWPVVWAVLQLGWRPGWFLDSPDRPWNPPTFSPALLVVTEGDNATFTCSFSNTSESFVLNWYRMSPSNQTDKLAAFPEDRSQPGQDCRFRVTQLPNGRDFHMSVVRARRNDSGTYLCGAISLAPKAQIKESLRAELRVTERRAEGGGGSGGGGSDKTHTCPPCPAPELLGGPSVFLFPPKPKDTLMISRTPEVTCVVVDVSHEDPEVKFNWYVDGVEVHNAKTKPREEQYNSTYRVVSVLTVLHRDWLNGKEYKCKVSNKALPAPIEKTISKAKGQPREPQVYTLPPSRDELTKNQVSLTCLVKGFYPSDIAVEWESNGQPENNYKTTPPVLDSDGSFFLYSKLTVDKSRWQQGNVFSCSVLHEALHNHYTQKSLSLSPGGGGGSHKSSSQGQDRHMIRMRQLIDIVDQLKNYVNDLVPEFLPAPEDVETNCEWSAFSCFQKAQLKSANTGNNERIINVSIKKLKRKPPSTNAGRRQKHRLTCPSCDSYEKKPPKEFLERFKSLLQKMIHQHLSSRTHGSEDS

SEQ ID NO: 8 - protein, 505 aa, synthetic construct
  REGION 1..505: note = hPD-1 D-Fc(29)-hIL-21
LDSPDRPWNPPTFSPALLVVTEGDNATFTCSFSNTSESFVLNWYRMSPSNQTDKLAAFPEDRSQPGQDCRFRVTQLPNGRDFHMSVVRARRNDSGTYLCGAISLAPKAQIKESLRAELRVTERRAEGGGGSGGGGSDKTHTCPPCPAPELLGGPSVFLFPPKPKDTLMISRTPEVTCVVVDVSHEDPEVKFNWYVDGVEVHNAKTKPREEQYNSTYRVVSVLTVLHRDWLNGKEYKCKVSNKALPAPIEKTISKAKGQPREPQVYTLPPSRDELTKNQVSLTCLVKGFYPSDIAVEWESNGQPENNYKTTPPVLDSDGSFFLYSKLTVDKSRWQQGNVFSCSVLHEALHNHYTQKSLSLSPGGGGGSHKSSSQGQDRHMIRMRQLIDIVDQLKNYVNDLVPEFLPAPEDVETNCEWSAFSCFQKAQLKSANTGNNERIINVSIKKLKRKPPSTNAGRRQKHRLTCPSCDSYEKKPPKEFLERFKSLLQKMIHQHLSSRTHGSEDS

SEQ ID NO: 9 - DNA, 1590 bp, synthetic construct
  misc_feature 1..1590: note = hPD-1 D-Fc(29)-hIL-21 Polynucleotide
  source 1..1590: mol_type = other DNA
atgcagatccctcaggctccatggccagtggtgtgggccgtgctccagctgggatggaggccaggctggttcctggactcccctgatcggccatggaatccccctacctttagcccagccctgctggtggtgacagagggcgacaacgctaccttcacatgctctttttccaacaccagcgagtctttcgtgctgaattggtacaggatgtcccccagcaaccagacagataagctggccgcttttccagaggaccggagccagcctggccaggattgcagattccgcgtgacccagctgcctaatggcagggactttcacatgtctgtggtgcgggccaggaggaacgattccggcacatacctgtgcggcgctatcagcctggccccaaaggctcagatcaaggagtccctgagagctgagctgagggtgaccgagagaagggctgagggaggaggaggctccggcggaggaggcagcgacaagacccatacatgcccaccatgtcctgctccagagctgctgggcggacctagcgtgttcctgtttcctccaaagccaaaggataccctgatgatctctaggaccccagaggtgacatgcgtggtggtggacgtgtcccacgaggaccccgaggtgaagttcaattggtacgtggacggcgtggaggtgcataacgctaagacaaagcccagagaggagcagtacaactctacctatcgcgtggtgtccgtgctgacagtgctgcacagagattggctgaatggcaaggagtataagtgcaaggtgagcaacaaggccctgcccgctcctatcgagaagaccatctctaaggccaagggccagcccagagagcctcaggtgtacacactgcccccttccagggacgagctgaccaagaatcaggtgtccctgacatgtctggtgaagggcttctatccctccgacatcgctgtggagtgggagagcaacggccagcctgagaacaattacaagaccacaccacccgtgctggacagcgatggctctttctttctgtatagcaagctgaccgtggacaagtccaggtggcagcagggcaacgtgttctcctgctccgtgctgcatgaggccctgcacaaccattacacacagaagagcctgtctctgtcccccggcggaggaggaggctctcacaagtccagctctcagggccaggatcgccacatgatcaggatgcggcagctgatcgacatcgtggatcagctgaagaactatgtgaatgacctggtgcctgagtttctgccagcccccgaggatgtggagaccaattgcgagtggtccgctttcagctgttttcagaaggcccagctgaagtctgctaatacaggcaacaatgagaggatcatcaacgtgagcatcaagaagctgaagcggaagcctccatctaccaacgctggcaggcggcagaagcacaggctgacatgcccttcttgtgactcctacgagaagaagccccctaaggagttcctggagaggttcaagtccctgctccagaagatgatccaccagcatctgtccagccgcacccatggcagcgaggattcttga

SEQ ID NO: 10 - protein, 216 aa, synthetic construct
  REGION 1..216: note = Fc(41)
APELLGGPSVFLFPPKPKDTLMISRTPEVTCVVVDVSHEDPEVKFNWYVDGVEVHNAKTKPREEQYNSTYRVVSVLTVGHQDWLNGKEYKCKVSNKALPAPIEKTISKAKGQPREPQVYTLPPSRDELTKNQVSLTCLVKGFYPSDIAVEWESNGQPENNYKTTPPVLDSDGSFFLYSKLTVDKSRWQQGNVFSCSVLHEALHNHYTQKSLSLSPG

SEQ ID NO: 11 - protein, 529 aa, synthetic construct
  REGION 1..529: note = hPD-1 D-Fc(41)-hIL-21 with signal peptide
MQIPQAPWPVVWAVLQLGWRPGWFLDSPDRPWNPPTFSPALLVVTEGDNATFTCSFSNTSESFVLNWYRMSPSNQTDKLAAFPEDRSQPGQDCRFRVTQLPNGRDFHMSVVRARRNDSGTYLCGAISLAPKAQIKESLRAELRVTERRAEGGGGSGGGGSDKTHTCPPCPAPELLGGPSVFLFPPKPKDTLMISRTPEVTCVVVDVSHEDPEVKFNWYVDGVEVHNAKTKPREEQYNSTYRVVSVLTVGHQDWLNGKEYKCKVSNKALPAPIEKTISKAKGQPREPQVYTLPPSRDELTKNQVSLTCLVKGFYPSDIAVEWESNGQPENNYKTTPPVLDSDGSFFLYSKLTVDKSRWQQGNVFSCSVLHEALHNHYTQKSLSLSPGGGGGSHKSSSQGQDRHMIRMRQLIDIVDQLKNYVNDLVPEFLPAPEDVETNCEWSAFSCFQKAQLKSANTGNNERIINVSIKKLKRKPPSTNAGRRQKHRLTCPSCDSYEKKPPKEFLERFKSLLQKMIHQHLSSRTHGSEDS

SEQ ID NO: 12 - protein, 505 aa, synthetic construct
  REGION 1..505: note = hPD-1 D-Fc(41)-hIL-21
LDSPDRPWNPPTFSPALLVVTEGDNATFTCSFSNTSESFVLNWYRMSPSNQTDKLAAFPEDRSQPGQDCRFRVTQLPNGRDFHMSVVRARRNDSGTYLCGAISLAPKAQIKESLRAELRVTERRAEGGGGSGGGGSDKTHTCPPCPAPELLGGPSVFLFPPKPKDTLMISRTPEVTCVVVDVSHEDPEVKFNWYVDGVEVHNAKTKPREEQYNSTYRVVSVLTVGHQDWLNGKEYKCKVSNKALPAPIEKTISKAKGQPREPQVYTLPPSRDELTKNQVSLTCLVKGFYPSDIAVEWESNGQPENNYKTTPPVLDSDGSFFLYSKLTVDKSRWQQGNVFSCSVLHEALHNHYTQKSLSLSPGGGGGSHKSSSQGQDRHMIRMRQLIDIVDQLKNYVNDLVPEFLPAPEDVETNCEWSAFSCFQKAQLKSANTGNNERIINVSIKKLKRKPPSTNAGRRQKHRLTCPSCDSYEKKPPKEFLERFKSLLQKMIHQHLSSRTHGSEDS

SEQ ID NO: 13 - DNA, 1590 bp, synthetic construct
  misc_feature 1..1590: note = hPD-1 D-Fc(41)-hIL-21 Polynucleotide
  source 1..1590: mol_type = other DNA
atgcagatccctcaggctccatggccagtggtgtgggccgtgctccagctgggatggaggccaggctggttcctggactcccctgatcggccatggaatccccctacctttagcccagccctgctggtggtgacagagggcgacaacgctaccttcacatgctctttttccaacaccagcgagtctttcgtgctgaattggtacaggatgtcccccagcaaccagacagataagctggccgcttttccagaggaccggagccagcctggccaggattgcagattccgcgtgacccagctgcctaatggcagggactttcacatgtctgtggtgcgggccaggaggaacgattccggcacatacctgtgcggcgctatcagcctggccccaaaggctcagatcaaggagtccctgagagctgagctgagggtgaccgagagaagggctgagggaggaggaggctccggcggaggaggcagcgacaagacccatacatgcccaccatgtcctgctccagagctgctgggcggacctagcgtgttcctgtttcctccaaagccaaaggataccctgatgatctctaggaccccagaggtgacatgcgtggtggtggacgtgtcccacgaggaccccgaggtgaagttcaattggtacgtggacggcgtggaggtgcataacgctaagacaaagcccagagaggagcagtacaactctacctatcgcgtggtgtccgtgctgacagtgggccaccaggattggctgaatggcaaggagtataagtgcaaggtgagcaacaaggccctgcccgctcctatcgagaagaccatctctaaggccaagggccagcccagagagcctcaggtgtacacactgcccccttccagggacgagctgaccaagaatcaggtgtccctgacatgtctggtgaagggcttctatccctccgacatcgctgtggagtgggagagcaacggccagcctgagaacaattacaagaccacaccacccgtgctggacagcgatggctctttctttctgtatagcaagctgaccgtggacaagtccaggtggcagcagggcaacgtgttctcctgctccgtgctgcatgaggccctgcacaaccattacacacagaagagcctgtctctgtcccccggcggaggaggaggctctcacaagtccagctctcagggccaggatcgccacatgatcaggatgcggcagctgatcgacatcgtggatcagctgaagaactatgtgaatgacctggtgcctgagtttctgccagcccccgaggatgtggagaccaattgcgagtggtccgctttcagctgttttcagaaggcccagctgaagtctgctaatacaggcaacaatgagaggatcatcaacgtgagcatcaagaagctgaagcggaagcctccatctaccaacgctggcaggcggcagaagcacagactgacatgcccttcttgtgactcctacgagaagaagccccctaaggagttcctggagaggttcaagtccctgctccagaagatgatccaccagcatctgtccagccgcacccatggcagcgaggattcttga

SEQ ID NO: 14 - protein, 216 aa, synthetic construct
  REGION 1..216: note = Fc(wt)
APELLGGPSVFLFPPKPKDTLMISRTPEVTCVVVDVSHEDPEVKFNWYVDGVEVHNAKTKPREEQYNSTYRVVSVLTVLHQDWLNGKEYKCKVSNKALPAPIEKTISKAKGQPREPQVYTLPPSRDELTKNQVSLTCLVKGFYPSDIAVEWESNGQPENNYKTTPPVLDSDGSFFLYSKLTVDKSRWQQGNVFSCSVMHEALHNHYTQKSLSLSPG

SEQ ID NO: 15 - protein, 529 aa, synthetic construct
  REGION 1..529: note = hPD-1 D-Fc(wt)-hIL-21 with signal peptide
MQIPQAPWPVVWAVLQLGWRPGWFLDSPDRPWNPPTFSPALLVVTEGDNATFTCSFSNTSESFVLNWYRMSPSNQTDKLAAFPEDRSQPGQDCRFRVTQLPNGRDFHMSVVRARRNDSGTYLCGAISLAPKAQIKESLRAELRVTERRAEGGGGSGGGGSDKTHTCPPCPAPELLGGPSVFLFPPKPKDTLMISRTPEVTCVVVDVSHEDPEVKFNWYVDGVEVHNAKTKPREEQYNSTYRVVSVLTVLHQDWLNGKEYKCKVSNKALPAPIEKTISKAKGQPREPQVYTLPPSRDELTKNQVSLTCLVKGFYPSDIAVEWESNGQPENNYKTTPPVLDSDGSFFLYSKLTVDKSRWQQGNVFSCSVMHEALHNHYTQKSLSLSPGGGGGSHKSSSQGQDRHMIRMRQLIDIVDQLKNYVNDLVPEFLPAPEDVETNCEWSAFSCFQKAQLKSANTGNNERIINVSIKKLKRKPPSTNAGRRQKHRLTCPSCDSYEKKPPKEFLERFKSLLQKMIHQHLSSRTHGSEDS

SEQ ID NO: 16 - protein, 505 aa, synthetic construct
  REGION 1..505: note = hPD-1 D-Fc(wt)-hIL-21
LDSPDRPWNPPTFSPALLVVTEGDNATFTCSFSNTSESFVLNWYRMSPSNQTDKLAAFPEDRSQPGQDCRFRVTQLPNGRDFHMSVVRARRNDSGTYLCGAISLAPKAQIKESLRAELRVTERRAEGGGGSGGGGSDKTHTCPPCPAPELLGGPSVFLFPPKPKDTLMISRTPEVTCVVVDVSHEDPEVKFNWYVDGVEVHNAKTKPREEQYNSTYRVVSVLTVLHQDWLNGKEYKCKVSNKALPAPIEKTISKAKGQPREPQVYTLPPSRDELTKNQVSLTCLVKGFYPSDIAVEWESNGQPENNYKTTPPVLDSDGSFFLYSKLTVDKSRWQQGNVFSCSVMHEALHNHYTQKSLSLSPGGGGGSHKSSSQGQDRHMIRMRQLIDIVDQLKNYVNDLVPEFLPAPEDVETNCEWSAFSCFQKAQLKSANTGNNERIINVSIKKLKRKPPSTNAGRRQKHRLTCPSCDSYEKKPPKEFLERFKSLLQKMIHQHLSSRTHGSEDS

SEQ ID NO: 17 - DNA, 1590 bp, synthetic construct
  misc_feature 1..1590: note = hPD-1 D-Fc(wt)-hIL-21 Polynucleotide
  source 1..1590: mol_type = other DNA
atgcagatccctcaggctccatggccagtggtgtgggccgtgctccagctgggatggaggccaggctggttcctggactcccctgatcggccatggaatccccctacctttagcccagccctgctggtggtgacagagggcgacaacgctaccttcacatgctctttttccaacaccagcgagtctttcgtgctgaattggtacaggatgtcccccagcaaccagacagataagctggccgcttttccagaggaccggagccagcctggccaggattgcagattccgcgtgacccagctgcctaatggcagggactttcacatgtctgtggtgcgggccaggaggaacgattccggcacatacctgtgcggcgctatcagcctggccccaaaggctcagatcaaggagtccctgagagctgagctgagggtgaccgagagaagggctgagggaggaggaggctccggcggaggaggcagcgacaagacccatacatgcccaccatgtcctgctccagagctgctgggcggacctagcgtgttcctgtttcctccaaagccaaaggataccctgatgatctctaggaccccagaggtgacatgcgtggtggtggacgtgtcccacgaggaccccgaggtgaagttcaattggtacgtggacggcgtggaggtgcataacgctaagacaaagcccagagaggagcagtacaactctacctatcgcgtggtgtccgtgctgacagtgctgcaccaggattggctgaatggcaaggagtataagtgcaaggtgagcaacaaggccctgcccgctcctatcgagaagaccatctctaaggccaagggccagcccagagagcctcaggtgtacacactgcccccttccagggacgagctgaccaagaatcaggtgtccctgacatgtctggtgaagggcttctatccctccgacatcgctgtggagtgggagagcaacggccagcctgagaacaattacaagaccacaccacccgtgctggacagcgatggctctttctttctgtatagcaagctgaccgtggacaagtccaggtggcagcagggcaacgtgttctcctgctccgtgatgcatgaggccctgcacaaccattacacacagaagagcctgtctctgtcccccggcggaggaggaggctctcacaagtccagctctcagggccaggatcgccacatgatcaggatgcggcagctgatcgacattgtggatcagctgaagaactatgtgaatgacctggtgcctgagtttctgccagcccccgaggatgtggagaccaattgcgagtggtccgctttcagctgttttcagaaggcccagctgaagtctgctaatacaggcaacaatgagaggatcatcaacgtgagcatcaagaagctgaagcggaagcctccatctaccaacgctggcaggcggcagaagcacagactgacatgcccttcttgtgactcctacgagaagaagccccctaaggagttcctggagaggttcaagtccctgctccagaagatgatccaccagcatctgtccagccgcacccatggcagcgaggattcttga

SEQ ID NO: 18 - protein, 288 aa, synthetic construct
  REGION 1..288: note = hPD-1 full length
MQIPQAPWPVVWAVLQLGWRPGWFLDSPDRPWNPPTFSPALLVVTEGDNATFTCSFSNTSESFVLNWYRMSPSNQTDKLAAFPEDRSQPGQDCRFRVTQLPNGRDFHMSVVRARRNDSGTYLCGAISLAPKAQIKESLRAELRVTERRAEVPTAHPSPSPRPAGQFQTLVVGVVGGLLGSLVLLVWVLAVICSRAARGTIGARRTGQPLKEDPSAVPVFSVDYGELDFQWREKTPEPPVPCVPEQTEYATIVFPSGMGTSSPARRGSADGPRSAQPLRPEDGHCSWPL

SEQ ID NO: 19 - protein, 162 aa, synthetic construct
  REGION 1..162: note = hIL-21 full length
MRSSPGNMERIVICLMVIFLGTLVHKSSSQGQDRHMIRMRQLIDIVDQLKNYVNDLVPEFLPAPEDVETNCEWSAFSCFQKAQLKSANTGNNERIINVSIKKLKRKPPSTNAGRRQKHRLTCPSCDSYEKKPPKEFLERFKSLLQKMIHQHLSSRTHGSEDS

SEQ ID NO: 20 - protein, 19 aa, synthetic construct
  REGION 1..19: note = Signal Peptide 2
MPRGWAAPLLLLLLQGGWG

SEQ ID NO: 21 - protein, 145 aa, synthetic construct
  REGION 1..145: note = mPD-1
LEVPNGPWRSLTFYPAWLTVSEGANATFTCSLSNWSEDLMLNWNRLSPSNQTEKQAAFCNGLSQPVQDARFQIIQLPNRHDFHMNILDTRRNDSGIYLCGAISLHPKAKIEESPGAELVVTERILETSTRYPSPSPKPEGRFQGM

SEQ ID NO: 22 - protein, 129 aa, synthetic construct
  REGION 1..129: note = mIL-21
HKSSPQGPDRLLIRLRHLIDIVEQLKIYENDLDPELLSAPQDVKGHCEHAAFACFQKAKLKPSNPGNNKTFIIDLVAQLRRRLPARRGGKKQKHIAKCPSCDSYEKRTPKEFLERLKWLLQKMIHQHLS

SEQ ID NO: 23 - protein, 534 aa, synthetic construct
  REGION 1..534: note = mPD-1 D-Fc(29)-mIL-21 with signal peptide
MPRGWAAPLLLLLLQGGWGLEVPNGPWRSLTFYPAWLTVSEGANATFTCSLSNWSEDLMLNWNRLSPSNQTEKQAAFCNGLSQPVQDARFQIIQLPNRHDFHMNILDTRRNDSGIYLCGAISLHPKAKIEESPGAELVVTERILETSTRYPSPSPKPEGRFQGMGGGGSGGGGSDKTHTCPPCPAPELLGGPSVFLFPPKPKDTLMISRTPEVTCVVVDVSHEDPEVKFNWYVDGVEVHNAKTKPREEQYNSTYRVVSVLTVLHRDWLNGKEYKCKVSNKALPAPIEKTISKAKGQPREPQVYTLPPSRDELTKNQVSLTCLVKGFYPSDIAVEWESNGQPENNYKTTPPVLDSDGSFFLYSKLTVDKSRWQQGNVFSCSVLHEALHNHYTQKSLSLSPGGGGGSHKSSPQGPDRLLIRLRHLIDIVEQLKIYENDLDPELLSAPQDVKGHCEHAAFACFQKAKLKPSNPGNNKTFIIDLVAQLRRRLPARRGGKKQKHIAKCPSCDSYEKRTPKEFLERLKWLLQKMIHQHLS

SEQ ID NO: 24 - protein, 515 aa, synthetic construct
  REGION 1..515: note = mPD-1 D-Fc(29)-mIL-21
LEVPNGPWRSLTFYPAWLTVSEGANATFTCSLSNWSEDLMLNWNRLSPSNQTEKQAAFCNGLSQPVQDARFQIIQLPNRHDFHMNILDTRRNDSGIYLCGAISLHPKAKIEESPGAELVVTERILETSTRYPSPSPKPEGRFQGMGGGGSGGGGSDKTHTCPPCPAPELLGGPSVFLFPPKPKDTLMISRTPEVTCVVVDVSHEDPEVKFNWYVDGVEVHNAKTKPREEQYNSTYRVVSVLTVLHRDWLNGKEYKCKVSNKALPAPIEKTISKAKGQPREPQVYTLPPSRDELTKNQVSLTCLVKGFYPSDIAVEWESNGQPENNYKTTPPVLDSDGSFFLYSKLTVDKSRWQQGNVFSCSVLHEALHNHYTQKSLSLSPGGGGGSHKSSPQGPDRLLIRLRHLIDIVEQLKIYENDLDPELLSAPQDVKGHCEHAAFACFQKAKLKPSNPGNNKTFIIDLVAQLRRRLPARRGGKKQKHIAKCPSCDSYEKRTPKEFLERLKWLLQKMIHQHLS

SEQ ID NO: 25 - DNA, 1605 bp, synthetic construct
  misc_feature 1..1605: note = mPD-1 D-Fc(29)-mIL-21 Polynucleotide
  source 1..1605: mol_type = other DNA
atgccacgcggctgggctgctccactgctgctgctgctgctccagggcggctggggcttggaagtccctaatggtccttggcgttcacttacattctaccccgcctggcttacagtgtcagagggtgcaaacgcaacatttacctgctccctttctaactggtctgaggacctcatgttgaactggaatcggctctcaccttccaatcaaaccgagaagcaagctgccttttgtaatgggcttagtcaacctgtacaggatgctcggtttcagattattcagctccctaatcgacatgactttcacatgaacatattggatacaagacggaatgatagtggaatatatctttgcggcgccatatctctgcaccctaaagctaagattgaggagtcaccaggggcagaactcgtggttaccgaacgcattctggaaacatcaaccaggtatccaagtccaagccccaaacccgagggcagattccagggcatgggaggaggaggctccggcggaggaggcagcgacaagacccatacatgcccaccatgtcctgctccagagctgctgggcggacctagcgtgttcctgtttcctccaaagccaaaggataccctgatgatctctaggaccccagaggtgacatgcgtggtggtggacgtgtcccacgaggaccccgaggtgaagttcaattggtacgtggacggcgtggaggtgcataacgctaagacaaagcccagagaggagcagtacaactctacctatcgcgtggtgtccgtgctgacagtgctgcacagagattggctgaatggcaaggagtataagtgcaaggtgagcaacaaggccctgcccgctcctatcgagaagaccatctctaaggccaagggccagcccagagagcctcaggtgtacacactgcccccttccagggacgagctgaccaagaatcaggtgtccctgacatgtctggtgaagggcttctatccctccgacatcgctgtggagtgggagagcaacggccagcctgagaacaattacaagaccacaccacccgtgctggacagcgatggctctttctttctgtatagcaagctgaccgtggacaagtccaggtggcagcagggcaacgtgttctcctgctccgtgctgcatgaggccctgcacaaccattacacacagaagagcctgtctctgtcccccggcggaggaggaggctctcataagagtagcccccaaggtccagacagactgcttatccgacttagacatctcatagacatcgttgagcaacttaaaatctatgaaaatgacctggaccctgagctgctgtctgctccacaggatgtaaagggtcactgcgaacatgctgctttcgcttgttttcagaaggcaaaactgaaaccatcaaatcccggcaataataagactttcattatagacctggttgctcaactgcgtcgaaggctccctgcacgacgaggtggtaagaaacaaaaacacatcgctaaatgccccagttgtgattcctatgagaagcgcacccctaaggagttcttggaaaggctcaagtggcttctccagaaaatgatccatcagcatctctcatga

SEQ ID NO: 26 - protein, 534 aa, synthetic construct
  REGION 1..534: note = mPD-1 D-Fc(wt)-mIL-21 with signal peptide
MPRGWAAPLLLLLLQGGWGLEVPNGPWRSLTFYPAWLTVSEGANATFTCSLSNWSEDLMLNWNRLSPSNQTEKQAAFCNGLSQPVQDARFQIIQLPNRHDFHMNILDTRRNDSGIYLCGAISLHPKAKIEESPGAELVVTERILETSTRYPSPSPKPEGRFQGMGGGGSGGGGSDKTHTCPPCPAPELLGGPSVFLFPPKPKDTLMISRTPEVTCVVVDVSHEDPEVKFNWYVDGVEVHNAKTKPREEQYNSTYRVVSVLTVLHQDWLNGKEYKCKVSNKALPAPIEKTISKAKGQPREPQVYTLPPSRDELTKNQVSLTCLVKGFYPSDIAVEWESNGQPENNYKTTPPVLDSDGSFFLYSKLTVDKSRWQQGNVFSCSVMHEALHNHYTQKSLSLSPGGGGGSHKSSPQGPDRLLIRLRHLIDIVEQLKIYENDLDPELLSAPQDVKGHCEHAAFACFQKAKLKPSNPGNNKTFIIDLVAQLRRRLPARRGGKKQKHIAKCPSCDSYEKRTPKEFLERLKWLLQKMIHQHLS

SEQ ID NO: 27 - protein, 515 aa, synthetic construct
  REGION 1..515: note = mPD-1 D-Fc(wt)-mIL-21
LEVPNGPWRSLTFYPAWLTVSEGANATFTCSLSNWSEDLMLNWNRLSPSNQTEKQAAFCNGLSQPVQDARFQIIQLPNRHDFHMNILDTRRNDSGIYLCGAISLHPKAKIEESPGAELVVTERILETSTRYPSPSPKPEGRFQGMGGGGSGGGGSDKTHTCPPCPAPELLGGPSVFLFPPKPKDTLMISRTPEVTCVVVDVSHEDPEVKFNWYVDGVEVHNAKTKPREEQYNSTYRVVSVLTVLHQDWLNGKEYKCKVSNKALPAPIEKTISKAKGQPREPQVYTLPPSRDELTKNQVSLTCLVKGFYPSDIAVEWESNGQPENNYKTTPPVLDSDGSFFLYSKLTVDKSRWQQGNVFSCSVMHEALHNHYTQKSLSLSPGGGGGSHKSSPQGPDRLLIRLRHLIDIVEQLKIYENDLDPELLSAPQDVKGHCEHAAFACFQKAKLKPSNPGNNKTFIIDLVAQLRRRLPARRGGKKQKHIAKCPSCDSYEKRTPKEFLERLKWLLQKMIHQHLS

SEQ ID NO: 28 - DNA, 1605 bp, synthetic construct
  misc_feature 1..1605: note = mPD-1 D-Fc(wt)-mIL-21 Polynucleotide
  source 1..1605: mol_type = other DNA
atgccacgcggctgggctgctccactgctgctgctgctgctccagggcggctggggcttggaagtccctaatggtccttggcgttcacttacattctaccccgcctggcttacagtgtcagagggtgcaaacgcaacatttacctgctccctttctaactggtctgaggacctcatgttgaactggaatcggctctcaccttccaatcaaaccgagaagcaagctgccttttgtaatgggcttagtcaacctgtacaggatgctcggtttcagattattcagctccctaatcgacatgactttcacatgaacatattggatacaagacggaatgatagtggaatatatctttgcggcgccatatctctgcaccctaaagctaagattgaggagtcaccaggggcagaactcgtggttaccgaacgcattctggaaacatcaaccaggtatccaagtccaagccccaaacccgagggcagattccagggcatgggaggaggaggctccggcggaggaggcagcgacaagacccatacatgcccaccatgtcctgctccagagctgctgggcggacctagcgtgttcctgtttcctccaaagccaaaggataccctgatgatctctaggaccccagaggtgacatgcgtggtggtggacgtgtcccacgaggaccccgaggtgaagttcaattggtacgtggacggcgtggaggtgcataacgctaagacaaagcccagagaggagcagtacaactctacctatcgcgtggtgtccgtgctgacagtgctgcaccaggattggctgaatggcaaggagtataagtgcaaggtgagcaacaaggccctgcccgctcctatcgagaagaccatctctaaggccaagggccagcccagagagcctcaggtgtacacactgcccccttccagggacgagctgaccaagaatcaggtgtccctgacatgtctggtgaagggcttctatccctccgacatcgctgtggagtgggagagcaacggccagcctgagaacaattacaagaccacaccacccgtgctggacagcgatggctctttctttctgtatagcaagctgaccgtggacaagtccaggtggcagcagggcaacgtgttctcctgctccgtgatgcatgaggccctgcacaaccattacacacagaagagcctgtctctgtcccccggcggaggaggaggctctcataagagtagcccccaaggtccagacagactgcttatccgacttagacatctcatagacatcgttgagcaacttaaaatctatgaaaatgacctggaccctgagctgctgtctgctccacaggatgtaaagggtcactgcgaacatgctgctttcgcttgttttcagaaggcaaaactgaaaccatcaaatcccggcaataataagactttcattatagacctggttgctcaactgcgtcgaaggctccctgcacgacgaggtggtaagaaacaaaaacacatcgctaaatgccccagttgtgattcctatgagaagcgcacccctaaggagttcttggaaaggctcaagtggcttctccagaaaatgatccatcagcatctctcatga

SEQ ID NO: 29 - protein, 288 aa, synthetic construct
  REGION 1..288: note = mPD-1 full length
MWVRQVPWSFTWAVLQLSWQSGWLLEVPNGPWRSLTFYPAWLTVSEGANATFTCSLSNWSEDLMLNWNRLSPSNQTEKQAAFCNGLSQPVQDARFQIIQLPNRHDFHMNILDTRRNDSGIYLCGAISLHPKAKIEESPGAELVVTERILETSTRYPSPSPKPEGRFQGMVIGIMSALVGIPVLLLLAWALAVFCSTSMSEARGAGSKDDTLKEEPSAAPVPSVAYEELDFQGREKTPELPTACVHTEYATIVFTEGLGASAMGRRGSADGLQGPRPPRHEDGHCSWPL

SEQ ID NO: 30 - protein, 146 aa, synthetic construct [sequence omitted]

SEQ ID NO: 31 - protein, 520 aa, synthetic construct
  REGION 1..520: note = hPD-1 D-Fc(29)-mIL-21 with signal peptide
MQIPQAPWPVVWAVLQLGWRPGWFLDSPDRPWNPPTFSPALLVVTEGDNATFTCSFSNTSESFVLNWYRMSPSNQTDKLAAFPEDRSQPGQDCRFRVTQLPNGRDFHMSVVRARRNDSGTYLCGAISLAPKAQIKESLRAELRVTERRAEGGGGSGGGGSDKTHTCPPCPAPELLGGPSVFLFPPKPKDTLMISRTPEVTCVVVDVSHEDPEVKFNWYVDGVEVHNAKTKPREEQYNSTYRVVSVLTVLHRDWLNGKEYKCKVSNKALPAPIEKTISKAKGQPREPQVYTLPPSRDELTKNQVSLTCLVKGFYPSDIAVEWESNGQPENNYKTTPPVLDSDGSFFLYSKLTVDKSRWQQGNVFSCSVLHEALHNHYTQKSLSLSPGGGGGSHKSSPQGPDRLLIRLRHLIDIVEQLKIYENDLDPELLSAPQDVKGHCEHAAFACFQKAKLKPSNPGNNKTFIIDLVAQLRRRLPARRGGKKQKHIAKCPSCDSYEKRTPKEFLERLKWLLQKMIHQHLS

SEQ ID NO: 32 - protein, 496 aa, synthetic construct
  REGION 1..496: note = hPD-1 D-Fc(29)-mIL-21
LDSPDRPWNPPTFSPALLVVTEGDNATFTCSFSNTSESFVLNWYRMSPSNQTDKLAAFPEDRSQPGQDCRFRVTQLPNGRDFHMSVVRARRNDSGTYLCGAISLAPKAQIKESLRAELRVTERRAEGGGGSGGGGSDKTHTCPPCPAPELLGGPSVFLFPPKPKDTLMISRTPEVTCVVVDVSHEDPEVKFNWYVDGVEVHNAKTKPREEQYNSTYRVVSVLTVLHRDWLNGKEYKCKVSNKALPAPIEKTISKAKGQPREPQVYTLPPSRDELTKNQVSLTCLVKGFYPSDIAVEWESNGQPENNYKTTPPVLDSDGSFFLYSKLTVDKSRWQQGNVFSCSVLHEALHNHYTQKSLSLSPGGGGGSHKSSPQGPDRLLIRLRHLIDIVEQLKIYENDLDPELLSAPQDVKGHCEHAAFACFQKAKLKPSNPGNNKTFIIDLVAQLRRRLPARRGGKKQKHIAKCPSCDSYEKRTPKEFLERLKWLLQKMIHQHLS

SEQ ID NO: 33 - DNA, 1563 bp, synthetic construct
  misc_feature 1..1563: note = hPD-1 D-Fc(29)-mIL-21 Polynucleotide
  source 1..1563: mol_type = other DNA
atgcagatccctcaggctccatggccagtggtgtgggccgtgctccagctgggatggaggccaggctggttcctggactcccctgatcggccatggaatccccctacctttagcccagccctgctggtggtgacagagggcgacaacgctaccttcacatgctctttttccaacaccagcgagtctttcgtgctgaattggtacaggatgtcccccagcaaccagacagataagctggccgcttttccagaggaccggagccagcctggccaggattgcagattccgcgtgacccagctgcctaatggcagggactttcacatgtctgtggtgcgggccaggaggaacgattccggcacatacctgtgcggcgctatcagcctggccccaaaggctcagatcaaggagtccctgagagctgagctgagggtgaccgagagaagggctgagggaggaggaggctccggcggaggaggcagcgacaagacccatacatgcccaccatgtcctgctccagagctgctgggcggacctagcgtgttcctgtttcctccaaagccaaaggataccctgatgatctctaggaccccagaggtgacatgcgtggtggtggacgtgtcccacgaggaccccgaggtgaagttcaattggtacgtggacggcgtggaggtgcataacgctaagacaaagcccagagaggagcagtacaactctacctatcgcgtggtgtccgtgctgacagtgctgcacagagattggctgaatggcaaggagtataagtgcaaggtgagcaacaaggccctgcccgctcctatcgagaagaccatctctaaggccaagggccagcccagagagcctcaggtgtacacactgcccccttccagggacgagctgaccaagaatcaggtgtccctgacatgtctggtgaagggcttctatccctccgacatcgctgtggagtgggagagcaacggccagcctgagaacaattacaagaccacaccacccgtgctggacagcgatggctctttctttctgtatagcaagctgaccgtggacaagtccaggtggcagcagggcaacgtgttctcctgctccgtgctgcatgaggccctgcacaaccattacacacagaagagcctgtctctgtcccccggcggaggaggaggctctcataagagtagcccccaaggtccagacagactgcttatccgacttagacatctcatagacatcgttgagcaacttaaaatctatgaaaatgacctggaccctgagctgctgtctgctccacaggatgtaaagggtcactgcgaacatgctgctttcgcttgttttcagaaggcaaaactgaaaccatcaaatcccggcaataataagactttcattatagacctggttgctcaactgcgtcgaaggctccctgcacgacgaggtggtaagaaacaaaaacacatcgctaaatgccccagttgtgattcctatgagaagcgcacccctaaggagttcttggaaaggctcaagtggcttctccagaaaatgatccatcagcatctctcatga

SEQ ID NO: 34 - protein, 146 aa, synthetic construct [sequence omitted]

SEQ ID NO: 35 - protein, 549 aa, synthetic construct
  REGION 1..549: note = hPD-1 ECD-Fc(29)-hIL-21 with signal peptide
MQIPQAPWPVVWAVLQLGWRPGWFLDSPDRPWNPPTFSPALLVVTEGDNATFTCSFSNTSESFVLNWYRMSPSNQTDKLAAFPEDRSQPGQDCRFRVTQLPNGRDFHMSVVRARRNDSGTYLCGAISLAPKAQIKESLRAELRVTERRAEVPTAHPSPSPRPAGQFQTLVGGGGSGGGGSDKTHTCPPCPAPELLGGPSVFLFPPKPKDTLMISRTPEVTCVVVDVSHEDPEVKFNWYVDGVEVHNAKTKPREEQYNSTYRVVSVLTVLHRDWLNGKEYKCKVSNKALPAPIEKTISKAKGQPREPQVYTLPPSRDELTKNQVSLTCLVKGFYPSDIAVEWESNGQPENNYKTTPPVLDSDGSFFLYSKLTVDKSRWQQGNVFSCSVLHEALHNHYTQKSLSLSPGGGGGSHKSSSQGQDRHMIRMRQLIDIVDQLKNYVNDLVPEFLPAPEDVETNCEWSAFSCFQKAQLKSANTGNNERIINVSIKKLKRKPPSTNAGRRQKHRLTCPSCDSYEKKPPKEFLERFKSLLQKMIHQHLSSRTHGSEDS

SEQ ID NO: 36 - protein, 525 aa, synthetic construct
  REGION 1..525: note = hPD-1 ECD-Fc(29)-hIL-21
LDSPDRPWNPPTFSPALLVVTEGDNATFTCSFSNTSESFVLNWYRMSPSNQTDKLAAFPEDRSQPGQDCRFRVTQLPNGRDFHMSVVRARRNDSGTYLCGAISLAPKAQIKESLRAELRVTERRAEVPTAHPSPSPRPAGQFQTLVGGGGSGGGGSDKTHTCPPCPAPELLGGPSVFLFPPKPKDTLMISRTPEVTCVVVDVSHEDPEVKFNWYVDGVEVHNAKTKPREEQYNSTYRVVSVLTVLHRDWLNGKEYKCKVSNKALPAPIEKTISKAKGQPREPQVYTLPPSRDELTKNQVSLTCLVKGFYPSDIAVEWESNGQPENNYKTTPPVLDSDGSFFLYSKLTVDKSRWQQGNVFSCSVLHEALHNHYTQKSLSLSPGGGGGSHKSSSQGQDRHMIRMRQLIDIVDQLKNYVNDLVPEFLPAPEDVETNCEWSAFSCFQKAQLKSANTGNNERIINVSIKKLKRKPPSTNAGRRQKHRLTCPSCDSYEKKPPKEFLERFKSLLQKMIHQHLSSRTHGSEDS

SEQ ID NO: 37 - DNA, 1650 bp, synthetic construct
  misc_feature 1..1650: note = hPD-1 ECD-Fc(29)-hIL-21 Polynucleotide
  source 1..1650: mol_type = other DNA
atgcagatccctcaggctccatggccagtggtgtgggccgtgctccagctgggatggaggccaggctggttcctggactcccctgatcggccatggaatccccctacctttagcccagccctgctggtggtgacagagggcgacaacgctaccttcacatgctctttttccaacaccagcgagtctttcgtgctgaattggtacaggatgtcccccagcaaccagacagataagctggccgcttttccagaggaccggagccagcctggccaggattgcagattccgcgtgacccagctgcctaatggcagggactttcacatgtctgtggtgcgggccaggaggaacgattccggcacatacctgtgcggcgctatcagcctggccccaaaggctcagatcaaggagtccctgagagctgagctgagggtgaccgagagaagggctgaggttccaactgctcatccctctcctagcccccgccctgccggccaattccaaacactggtaggaggaggaggctccggcggaggaggcagcgacaagacccatacatgcccaccatgtcctgctccagagctgctgggcggacctagcgtgttcctgtttcctccaaagccaaaggataccctgatgatctctaggaccccagaggtgacatgcgtggtggtggacgtgtcccacgaggaccccgaggtgaagttcaattggtacgtggacggcgtggaggtgcataacgctaagacaaagcccagagaggagcagtacaactctacctatcgcgtggtgtccgtgctgacagtgctgcacagagattggctgaatggcaaggagtataagtgcaaggtgagcaacaaggccctgcccgctcctatcgagaagaccatctctaaggccaagggccagcccagagagcctcaggtgtacacactgcccccttccagggacgagctgaccaagaatcaggtgtccctgacatgtctggtgaagggcttctatccctccgacatcgctgtggagtgggagagcaacggccagcctgagaacaattacaagaccacaccacccgtgctggacagcgatggctctttctttctgtatagcaagctgaccgtggacaagtccaggtggcagcagggcaacgtgttctcctgctccgtgctgcatgaggccctgcacaaccattacacacagaagagcctgtctctgtcccccggcggaggaggaggctctcacaagtccagctctcagggccaggatcgccacatgatcaggatgcggcagctgatcgacatcgtggatcagctgaagaactatgtgaatgacctggtgcctgagtttctgccagcccccgaggatgtggagaccaattgcgagtggtccgctttcagctgttttcagaaggcccagctgaagtctgctaatacaggcaacaatgagaggatcatcaacgtgagcatcaagaagctgaagcggaagcctccatctaccaacgctggcaggcggcagaagcacaggctgacatgcccttcttgtgactcctacgagaagaagccccctaaggagttcctggagaggttcaagtccctgctccagaagatgatccaccagcatctgtccagccgcacccatggcagcgaggattcttga

SEQ ID NO: 38 - protein, 15 aa, synthetic construct
  REGION 1..15: note = Hinge with linker 2
GGGGSDKTHTCPPCP

SEQ ID NO: 39 - protein, 20 aa, synthetic construct
  REGION 1..20: note = Linker 2
GGGGSGGGGSGGGGSGGGGS

SEQ ID NO: 40 - protein, 534 aa, synthetic construct
  REGION 1..534: note = hIL-21_Fc(29)_hPD-1 D with signal peptide
MPRGWAAPLLLLLLQGGWGHKSSSQGQDRHMIRMRQLIDIVDQLKNYVNDLVPEFLPAPEDVETNCEWSAFSCFQKAQLKSANTGNNERIINVSIKKLKRKPPSTNAGRRQKHRLTCPSCDSYEKKPPKEFLERFKSLLQKMIHQHLSSRTHGSEDSGGGGSDKTHTCPPCPAPELLGGPSVFLFPPKPKDTLMISRTPEVTCVVVDVSHEDPEVKFNWYVDGVEVHNAKTKPREEQYNSTYRVVSVLTVLHRDWLNGKEYKCKVSNKALPAPIEKTISKAKGQPREPQVYTLPPSRDELTKNQVSLTCLVKGFYPSDIAVEWESNGQPENNYKTTPPVLDSDGSFFLYSKLTVDKSRWQQGNVFSCSVLHEALHNHYTQKSLSLSPGGGGGSGGGGSGGGGSGGGGSLDSPDRPWNPPTFSPALLVVTEGDNATFTCSFSNTSESFVLNWYRMSPSNQTDKLAAFPEDRSQPGQDCRFRVTQLPNGRDFHMSVVRARRNDSGTYLCGAISLAPKAQIKESLRAELRVTERRAE

SEQ ID NO: 41 - protein, 515 aa, synthetic construct
  REGION 1..515: note = hIL-21_Fc(29)_hPD-1 D
HKSSSQGQDRHMIRMRQLIDIVDQLKNYVNDLVPEFLPAPEDVETNCEWSAFSCFQKAQLKSANTGNNERIINVSIKKLKRKPPSTNAGRRQKHRLTCPSCDSYEKKPPKEFLERFKSLLQKMIHQHLSSRTHGSEDSGGGGSDKTHTCPPCPAPELLGGPSVFLFPPKPKDTLMISRTPEVTCVVVDVSHEDPEVKFNWYVDGVEVHNAKTKPREEQYNSTYRVVSVLTVLHRDWLNGKEYKCKVSNKALPAPIEKTISKAKGQPREPQVYTLPPSRDELTKNQVSLTCLVKGFYPSDIAVEWESNGQPENNYKTTPPVLDSDGSFFLYSKLTVDKSRWQQGNVFSCSVLHEALHNHYTQKSLSLSPGGGGGSGGGGSGGGGSGGGGSLDSPDRPWNPPTFSPALLVVTEGDNATFTCSFSNTSESFVLNWYRMSPSNQTDKLAAFPEDRSQPGQDCRFRVTQLPNGRDFHMSVVRARRNDSGTYLCGAISLAPKAQIKESLRAELRVTERRAE

SEQ ID NO: 42 - DNA, 1605 bp, synthetic construct
  misc_feature 1..1605: note = hIL-21_Fc(29)_hPD-1 D Polynucleotide
  source 1..1605: mol_type = other DNA
atgccacgcggctgggctgctccactgctgctgctgctgctccagggcggctggggccacaagtccagctctcagggccaggatcgccacatgatcaggatgcggcagctgatcgacatcgtggatcagctgaagaactatgtgaatgacctggtgcctgagtttctgccagcccccgaggatgtggagaccaattgcgagtggtccgctttcagctgttttcagaaggcccagctgaagtctgctaatacaggcaacaatgagaggatcatcaacgtgagcatcaagaagctgaagcggaagcctccatctaccaacgctggcaggcggcagaagcacaggctgacatgcccttcttgtgactcctacgagaagaagccccctaaggagttcctggagaggttcaagtccctgctccagaagatgatccaccagcatctgtccagccgcacccatggcagcgaggattctggcggaggaggcagcgacaagacccatacatgcccaccatgtcctgctccagagctgctgggcggacctagcgtgttcctgtttcctccaaagccaaaggataccctgatgatctctaggaccccagaggtgacatgcgtggtggtggacgtgtcccacgaggaccccgaggtgaagttcaattggtacgtggacggcgtggaggtgcataacgctaagacaaagcccagagaggagcagtacaactctacctatcgcgtggtgtccgtgctgacagtgctgcacagagattggctgaatggcaaggagtataagtgcaaggtgagcaacaaggccctgcccgctcctatcgagaagaccatctctaaggccaagggccagcccagagagcctcaggtgtacacactgcccccttccagggacgagctgaccaagaatcaggtgtccctgacatgtctggtgaagggcttctatccctccgacatcgctgtggagtgggagagcaacggccagcctgagaacaattacaagaccacaccacccgtgctggacagcgatggctctttctttctgtatagcaagctgaccgtggacaagtccaggtggcagcagggcaacgtgttctcctgctccgtgctgcatgaggccctgcacaaccattacacacagaagagcctgtctctgtcccccggcggaggaggaggctctggaggcggaggatccggaggtgggggaagcggtggtggtggcagcctggactcccctgatcggccatggaatccccctacctttagcccagccctgctggtggtgacagagggcgacaacgctaccttcacatgctctttttccaacaccagcgagtctttcgtgctgaattggtacaggatgtcccccagcaaccagacagataagctggccgcttttccagaggaccggagccagcctggccaggattgcagattccgcgtgacccagctgcctaatggcagggactttcacatgtctgtggtgcgggccaggaggaacgattccggcacatacctgtgcggcgctatcagcctggccccaaaggctcagatcaaggagtccctgagagctgagctgagggtgaccgagagaagggctgagtga

SEQ ID NO: 43 - protein, 554 aa, synthetic construct
  REGION 1..554: note = hIL-21_Fc(29)_hPD-1 ECD with signal peptide
MPRGWAAPLLLLLLQGGWGHKSSSQGQDRHMIRMRQLIDIVDQLKNYVNDLVPEFLPAPEDVETNCEWSAFSCFQKAQLKSANTGNNERIINVSIKKLKRKPPSTNAGRRQKHRLTCPSCDSYEKKPPKEFLERFKSLLQKMIHQHLSSRTHGSEDSGGGGSDKTHTCPPCPAPELLGGPSVFLFPPKPKDTLMISRTPEVTCVVVDVSHEDPEVKFNWYVDGVEVHNAKTKPREEQYNSTYRVVSVLTVLHRDWLNGKEYKCKVSNKALPAPIEKTISKAKGQPREPQVYTLPPSRDELTKNQVSLTCLVKGFYPSDIAVEWESNGQPENNYKTTPPVLDSDGSFFLYSKLTVDKSRWQQGNVFSCSVLHEALHNHYTQKSLSLSPGGGGGSGGGGSGGGGSGGGGSLDSPDRPWNPPTFSPALLVVTEGDNATFTCSFSNTSESFVLNWYRMSPSNQTDKLAAFPEDRSQPGQDCRFRVTQLPNGRDFHMSVVRARRNDSGTYLCGAISLAPKAQIKESLRAELRVTERRAEVPTAHPSPSPRPAGQFQTLV

SEQ ID NO: 44 - protein, 535 aa, synthetic construct
  REGION 1..535: note = hIL-21_Fc(29)_hPD-1 ECD
HKSSSQGQDRHMIRMRQLIDIVDQLKNYVNDLVPEFLPAPEDVETNCEWSAFSCFQKAQLKSANTGNNERIINVSIKKLKRKPPSTNAGRRQKHRLTCPSCDSYEKKPPKEFLERFKSLLQKMIHQHLSSRTHGSEDSGGGGSDKTHTCPPCPAPELLGGPSVFLFPPKPKDTLMISRTPEVTCVVVDVSHEDPEVKFNWYVDGVEVHNAKTKPREEQYNSTYRVVSVLTVLHRDWLNGKEYKCKVSNKALPAPIEKTISKAKGQPREPQVYTLPPSRDELTKNQVSLTCLVKGFYPSDIAVEWESNGQPENNYKTTPPVLDSDGSFFLYSKLTVDKSRWQQGNVFSCSVLHEALHNHYTQKSLSLSPGGGGGSGGGGSGGGGSGGGGSLDSPDRPWNPPTFSPALLVVTEGDNATFTCSFSNTSESFVLNWYRMSPSNQTDKLAAFPEDRSQPGQDCRFRVTQLPNGRDFHMSVVRARRNDSGTYLCGAISLAPKAQIKESLRAELRVTERRAEVPTAHPSPSPRPAGQFQTLV

SEQ ID NO: 45 - DNA, 1665 bp, synthetic construct
  misc_feature 1..1665: note = hIL-21_Fc(29)_hPD-1 ECD Polynucleotide
  source 1..1665: mol_type = other DNA
atgccacgcggctgggctgctccactgctgctgctgctgctccagggcggctggggccacaagtccagctctcagggccaggatcgccacatgatcaggatgcggcagctgatcgacatcgtggatcagctgaagaactatgtgaatgacctggtgcctgagtttctgccagcccccgaggatgtggagaccaattgcgagtggtccgctttcagctgttttcagaaggcccagctgaagtctgctaatacaggcaacaatgagaggatcatcaacgtgagcatcaagaagctgaagcggaagcctccatctaccaacgctggcaggcggcagaagcacaggctgacatgcccttcttgtgactcctacgagaagaagccccctaaggagttcctggagaggttcaagtccctgctccagaagatgatccaccagcatctgtccagccgcacccatggcagcgaggattctggcggaggaggcagcgacaagacccatacatgcccaccatgtcctgctccagagctgctgggcggacctagcgtgttcctgtttcctccaaagccaaaggataccctgatgatctctaggaccccagaggtgacatgcgtggtggtggacgtgtcccacgaggaccccgaggtgaagttcaattggtacgtggacggcgtggaggtgcataacgctaagacaaagcccagagaggagcagtacaactctacctatcgcgtggtgtccgtgctgacagtgctgcacagagattggctgaatggcaaggagtataagtgcaaggtgagcaacaaggccctgcccgctcctatcgagaagaccatctctaaggccaagggccagcccagagagcctcaggtgtacacactgcccccttccagggacgagctgaccaagaatcaggtgtccctgacatgtctggtgaagggcttctatccctccgacatcgctgtggagtgggagagcaacggccagcctgagaacaattacaagaccacaccacccgtgctggacagcgatggctctttctttctgtatagcaagctgaccgtggacaagtccaggtggcagcagggcaacgtgttctcctgctccgtgctgcatgaggccctgcacaaccattacacacagaagagcctgtctctgtcccccggcggaggaggaggctctggaggcggaggatccggaggtgggggaagcggtggtggtggcagcctggactcccctgatcggccatggaatccccctacctttagcccagccctgctggtggtgacagagggcgacaacgctaccttcacatgctctttttccaacaccagcgagtctttcgtgctgaattggtacaggatgtcccccagcaaccagacagataagctggccgcttttccagaggaccggagccagcctggccaggattgcagattccgcgtgacccagctgcctaatggcagggactttcacatgtctgtggtgcgggccaggaggaacgattccggcacatacctgtgcggcgctatcagcctggccccaaaggctcagatcaaggagtccctgagagctgagctgagggtgaccgagagaagggctgaggttccaactgctcatccctctcctagcccccgccctgccggccaattccaaacactggtatga

SEQ ID NO: 46 - protein, 10 aa, synthetic construct
  REGION 1..10: note = Hinge
DKTHTCPPCP

SEQ ID NO: 47 - protein, 388 aa, synthetic construct
  REGION 1..388: note = Fc(29)_hIL-21 with signal peptide
MPRGWAAPLLLLLLQGGWGDKTHTCPPCPAPELLGGPSVFLFPPKPKDTLMISRTPEVTCVVVDVSHEDPEVKFNWYVDGVEVHNAKTKPREEQYNSTYRVVSVLTVLHRDWLNGKEYKCKVSNKALPAPIEKTISKAKGQPREPQVYTLPPSRDELTKNQVSLTCLVKGFYPSDIAVEWESNGQPENNYKTTPPVLDSDGSFFLYSKLTVDKSRWQQGNVFSCSVLHEALHNHYTQKSLSLSPGGGGGSHKSSSQGQDRHMIRMRQLIDIVDQLKNYVNDLVPEFLPAPEDVETNCEWSAFSCFQKAQLKSANTGNNERIINVSIKKLKRKPPSTNAGRRQKHRLTCPSCDSYEKKPPKEFLERFKSLLQKMIHQHLSSRTHGSEDS

SEQ ID NO: 48 - protein, 369 aa, synthetic construct
  REGION 1..369: note = Fc(29)_hIL-21
DKTHTCPPCPAPELLGGPSVFLFPPKPKDTLMISRTPEVTCVVVDVSHEDPEVKFNWYVDGVEVHNAKTKPREEQYNSTYRVVSVLTVLHRDWLNGKEYKCKVSNKALPAPIEKTISKAKGQPREPQVYTLPPSRDELTKNQVSLTCLVKGFYPSDIAVEWESNGQPENNYKTTPPVLDSDGSFFLYSKLTVDKSRWQQGNVFSCSVLHEALHNHYTQKSLSLSPGGGGGSHKSSSQGQDRHMIRMRQLIDIVDQLKNYVNDLVPEFLPAPEDVETNCEWSAFSCFQKAQLKSANTGNNERIINVSIKKLKRKPPSTNAGRRQKHRLTCPSCDSYEKKPPKEFLERFKSLLQKMIHQHLSSRTHGSEDS

SEQ ID NO: 49 - DNA, 1167 bp, synthetic construct
  misc_feature 1..1167: note = Fc(29)_hIL-21 Polynucleotide
  source 1..1167: mol_type = other DNA
atgccacgcggctgggctgctccactgctgctgctgctgctccagggcggctggggcgacaagacccatacatgcccaccatgtcctgctccagagctgctgggcggacctagcgtgttcctgtttcctccaaagccaaaggataccctgatgatctctaggaccccagaggtgacatgcgtggtggtggacgtgtcccacgaggaccccgaggtgaagttcaattggtacgtggacggcgtggaggtgcataacgctaagacaaagcccagagaggagcagtacaactctacctatcgcgtggtgtccgtgctgacagtgctgcacagagattggctgaatggcaaggagtataagtgcaaggtgagcaacaaggccctgcccgctcctatcgagaagaccatctctaaggccaagggccagcccagagagcctcaggtgtacacactgcccccttccagggacgagctgaccaagaatcaggtgtccctgacatgtctggtgaagggcttctatccctccgacatcgctgtggagtgggagagcaacggccagcctgagaacaattacaagaccacaccacccgtgctggacagcgatggctctttctttctgtatagcaagctgaccgtggacaagtccaggtggcagcagggcaacgtgttctcctgctccgtgctgcatgaggccctgcacaaccattacacacagaagagcctgtctctgtcccccggcggaggaggaggctctcacaagtccagctctcagggccaggatcgccacatgatcaggatgcggcagctgatcgacatcgtggatcagctgaagaactatgtgaatgacctggtgcctgagtttctgccagcccccgaggatgtggagaccaattgcgagtggtccgctttcagctgttttcagaaggcccagctgaagtctgctaatacaggcaacaatgagaggatcatcaacgtgagcatcaagaagctgaagcggaagcctccatctaccaacgctggcaggcggcagaagcacaggctgacatgcccttcttgtgactcctacgagaagaagccccctaaggagttcctggagaggttcaagtccctgctccagaagatgatccaccagcatctgtccagccgcacccatggcagcgaggattcttga

SEQ ID NO: 50 - protein, 216 aa, synthetic construct
  REGION 1..216: note = Fc(29, K)
APELLGGPSVFLFPPKPKDTLMISRTPEVTCVVVDVSHEDPEVKFNWYVDGVEVHNAKTKPREEQYNSTYRVVSVLTVLHRDWLNGKEYKCKVSNKALPAPIEKTISKAKGQPREPQVYTLPPSRDELTKNQVSLWCLVKGFYPSDIAVEWESNGQPENNYKTTPPVLDSDGSFFLYSKLTVDKSRWQQGNVFSCSVLHEALHNHYTQKSLSLSPG

SEQ ID NO: 51 - protein, 529 aa, synthetic construct
  REGION 1..529: note = hPD-1 D-Fc(29, K)-hIL-21 with signal peptide
MQIPQAPWPVVWAVLQLGWRPGWFLDSPDRPWNPPTFSPALLVVTEGDNATFTCSFSNTSESFVLNWYRMSPSNQTDKLAAFPEDRSQPGQDCRFRVTQLPNGRDFHMSVVRARRNDSGTYLCGAISLAPKAQIKESLRAELRVTERRAEGGGGSGGGGSDKTHTCPPCPAPELLGGPSVFLFPPKPKDTLMISRTPEVTCVVVDVSHEDPEVKFNWYVDGVEVHNAKTKPREEQYNSTYRVVSVLTVLHRDWLNGKEYKCKVSNKALPAPIEKTISKAKGQPREPQVYTLPPSRDELTKNQVSLWCLVKGFYPSDIAVEWESNGQPENNYKTTPPVLDSDGSFFLYSKLTVDKSRWQQGNVFSCSVLHEALHNHYTQKSLSLSPGGGGGSHKSSSQGQDRHMIRMRQLIDIVDQLKNYVNDLVPEFLPAPEDVETNCEWSAFSCFQKAQLKSANTGNNERIINVSIKKLKRKPPSTNAGRRQKHRLTCPSCDSYEKKPPKEFLERFKSLLQKMIHQHLSSRTHGSEDS

SEQ ID NO: 52 - protein, 505 aa, synthetic construct
  REGION 1..505: note = hPD-1 D-Fc(29, K)-hIL-21
LDSPDRPWNPPTFSPALLVVTEGDNATFTCSFSNTSESFVLNWYRMSPSNQTDKLAAFPEDRSQPGQDCRFRVTQLPNGRDFHMSVVRARRNDSGTYLCGAISLAPKAQIKESLRAELRVTERRAEGGGGSGGGGSDKTHTCPPCPAPELLGGPSVFLFPPKPKDTLMISRTPEVTCVVVDVSHEDPEVKFNWYVDGVEVHNAKTKPREEQYNSTYRVVSVLTVLHRDWLNGKEYKCKVSNKALPAPIEKTISKAKGQPREPQVYTLPPSRDELTKNQVSLWCLVKGFYPSDIAVEWESNGQPENNYKTTPPVLDSDGSFFLYSKLTVDKSRWQQGNVFSCSVLHEALHNHYTQKSLSLSPGGGGGSHKSSSQGQDRHMIRMRQLIDIVDQLKNYVNDLVPEFLPAPEDVETNCEWSAFSCFQKAQLKSANTGNNERIINVSIKKLKRKPPSTNAGRRQKHRLTCPSCDSYEKKPPKEFLERFKSLLQKMIHQHLSSRTHGSEDS

SEQ ID NO: 53 - DNA, 1590 bp, synthetic construct
  misc_feature 1..1590: note = hPD-1 D-Fc(29, K)-hIL-21 Polynucleotide
  source 1..1590: mol_type = other DNA
atgcagatccctcaggctccatggccagtggtgtgggccgtgctccagctgggatggaggccaggctggttcctggactcccctgatcggccatggaatccccctacctttagcccagccctgctggtggtgacagagggcgacaacgctaccttcacatgctctttttccaacaccagcgagtctttcgtgctgaattggtacaggatgtcccccagcaaccagacagataagctggccgcttttccagaggaccggagccagcctggccaggattgcagattccgcgtgacccagctgcctaatggcagggactttcacatgtctgtggtgcgggccaggaggaacgattccggcacatacctgtgcggcgctatcagcctggccccaaaggctcagatcaaggagtccctgagagctgagctgagggtgaccgagagaagggctgagggaggaggaggctccggcggaggaggcagcgacaagacccatacatgcccaccatgtcctgctccagagctgctgggcggacctagcgtgttcctgtttcctccaaagccaaaggataccctgatgatctctaggaccccagaggtgacatgcgtggtggtggacgtgtcccacgaggaccccgaggtgaagttcaattggtacgtggacggcgtggaggtgcataacgctaagacaaagcccagagaggagcagtacaactctacctatcgcgtggtgtccgtgctgacagtgctgcacagagattggctgaatggcaaggagtataagtgcaaggtgagcaacaaggccctgcccgctcctatcgagaagaccatctctaaggccaagggccagcccagagagcctcaggtgtacacactgcccccttccagggacgagctgaccaagaatcaggtgtccctgtggtgtctggtgaagggcttctatccctccgacatcgctgtggagtgggagagcaacggccagcctgagaacaattacaagaccacaccacccgtgctggacagcgatggctctttctttctgtatagcaagctgaccgtggacaagtccaggtggcagcagggcaacgtgttctcctgctccgtgctgcatgaggccctgcacaaccattacacacagaagagcctgtctctgtcccccggcggaggaggaggctctcacaagtccagctctcagggccaggatcgccacatgatcaggatgcggcagctgatcgacatcgtggatcagctgaagaactatgtgaatgacctggtgcctgagtttctgccagcccccgaggatgtggagaccaattgcgagtggtccgctttcagctgttttcagaaggcccagctgaagtctgctaatacaggcaacaatgagaggatcatcaacgtgagcatcaagaagctgaagcggaagcctccatctaccaacgctggcaggcggcagaagcacaggctgacatgcccttcttgtgactcctacgagaagaagccccctaaggagttcctggagaggttcaagtccctgctccagaagatgatccaccagcatctgtccagccgcacccatggcagcgaggattcttga

SEQ ID NO: 54 - protein, 520 aa, synthetic construct
  REGION 1..520: note = hPD-1 D-Fc(29, K)_mIL-21 with signal peptide
MQIPQAPWPVVWAVLQLGWRPGWFLDSPDRPWNPPTFSPALLVVTEGDNATFTCSFSNTSESFVLNWYRMSPSNQTDKLAAFPEDRSQPGQDCRFRVTQLPNGRDFHMSVVRARRNDSGTYLCGAISLAPKAQIKESLRAELRVTERRAEGGGGSGGGGSDKTHTCPPCPAPELLGGPSVFLFPPKPKDTLMISRTPEVTCVVVDVSHEDPEVKFNWYVDGVEVHNAKTKPREEQYNSTYRVVSVLTVLHRDWLNGKEYKCKVSNKALPAPIEKTISKAKGQPREPQVYTLPPSRDELTKNQVSLWCLVKGFYPSDIAVEWESNGQPENNYKTTPPVLDSDGSFFLYSKLTVDKSRWQQGNVFSCSVLHEALHNHYTQKSLSLSPGGGGGSHKSSPQGPDRLLIRLRHLIDIVEQLKIYENDLDPELLSAPQDVKGHCEHAAFACFQKAKLKPSNPGNNKTFIIDLVAQLRRRLPARRGGKKQKHIAKCPSCDSYEKRTPKEFLERLKWLLQKMIHQHLS

SEQ ID NO: 55 - protein, 496 aa, synthetic construct
  REGION 1..496: note = hPD-1 D-Fc(29, K)_mIL-21
LDSPDRPWNPPTFSPALLVVTEGDNATFTCSFSNTSESFVLNWYRMSPSNQTDKLAAFPEDRSQPGQDCRFRVTQLPNGRDFHMSVVRARRNDSGTYLCGAISLAPKAQIKESLRAELRVTERRAEGGGGSGGGGSDKTHTCPPCPAPELLGGPSVFLFPPKPKDTLMISRTPEVTCVVVDVSHEDPEVKFNWYVDGVEVHNAKTKPREEQYNSTYRVVSVLTVLHRDWLNGKEYKCKVSNKALPAPIEKTISKAKGQPREPQVYTLPPSRDELTKNQVSLWCLVKGFYPSDIAVEWESNGQPENNYKTTPPVLDSDGSFFLYSKLTVDKSRWQQGNVFSCSVLHEALHNHYTQKSLSLSPGGGGGSHKSSPQGPDRLLIRLRHLIDIVEQLKIYENDLDPELLSAPQDVKGHCEHAAFACFQKAKLKPSNPGNNKTFIIDLVAQLRRRLPARRGGKKQKHIAKCPSCDSYEKRTPKEFLERLKWLLQKMIHQHLS

SEQ ID NO: 56 - DNA, 1563 bp, synthetic construct
  misc_feature 1..1563: note = hPD-1 D-Fc(29, K)_mIL-21 Polynucleotide
  source 1..1563: mol_type = other DNA
atgcagatccctcaggctccatggccagtggtgtgggccgtgctccagctgggatggaggccaggctggttcctggactcccctgatcggccatggaatccccctacctttagcccagccctgctggtggtgacagagggcgacaacgctaccttcacatgctctttttccaacaccagcgagtctttcgtgctgaattggtacaggatgtcccccagcaaccagacagataagctggccgcttttccagaggaccggagccagcctggccaggattgcagattccgcgtgacccagctgcctaatggcagggactttcacatgtctgtggtgcgggccaggaggaacgattccggcacatacctgtgcggcgctatcagcctggccccaaaggctcagatcaaggagtccctgagagctgagctgagggtgaccgagagaagggctgagggaggaggaggctccggcggaggaggcagcgacaagacccatacatgcccaccatgtcctgctccagagctgctgggcggacctagcgtgttcctgtttcctccaaagccaaaggataccctgatgatctctaggaccccagaggtgacatgcgtggtggtggacgtgtcccacgaggaccccgaggtgaagttcaattggtacgtggacggcgtggaggtgcataacgctaagacaaagcccagagaggagcagtacaactctacctatcgcgtggtgtccgtgctgacagtgctgcacagagattggctgaatggcaaggagtataagtgcaaggtgagcaacaaggccctgcccgctcctatcgagaagaccatctctaaggccaagggccagcccagagagcctcaggtgtacacactgcccccttccagggacgagctgaccaagaatcaggtgtccctgtggtgtctggtgaagggcttctatccctccgacatcgctgtggagtgggagagcaacggccagcctgagaacaattacaagaccacaccacccgtgctggacagcgatggctctttctttctgtatagcaagctgaccgtggacaagtccaggtggcagcagggcaacgtgttctcctgctccgtgctgcatgaggccctgcacaaccattacacacagaagagcctgtctctgtcccccggcggaggaggaggctctcataagagtagcccccaaggtccagacagactgcttatccgacttagacatctcatagacatcgttgagcaacttaaaatctatgaaaatgacctggaccctgagctgctgtctgctccacaggatgtaaagggtcactgcgaacatgctgctttcgcttgttttcagaaggcaaaactgaaaccatcaaatcccggcaataataagactttcattatagacctggttgctcaactgcgtcgaaggctccctgcacgacgaggtggtaagaaacaaaaacacatcgctaaatgccccagttgtgattcctatgagaagcgcacccctaaggagttcttggaaaggctcaagtggcttctccagaaaatgatccatcagcatctctcatga

SEQ ID NO: 57 - protein, 15 aa, synthetic construct
  REGION 1..15: note = Linker 3
GGGGSGGGGSGGGGS

SEQ ID NO: 58 - protein, 6 aa, synthetic construct
  REGION 1..6: note = His tag
HHHHHH

SEQ ID NO: 59 - protein, 309 aa, synthetic construct
  REGION 1..309: note = hPD-1 D_hIL-21-6H with signal peptide
MQIPQAPWPVVWAVLQLGWRPGWFLDSPDRPWNPPTFSPALLVVTEGDNATFTCSFSNTSESFVLNWYRMSPSNQTDKLAAFPEDRSQPGQDCRFRVTQLPNGRDFHMSVVRARRNDSGTYLCGAISLAPKAQIKESLRAELRVTERRAEGGGGSGGGGSGGGGSHKSSSQGQDRHMIRMRQLIDIVDQLKNYVNDLVPEFLPAPEDVETNCEWSAFSCFQKAQLKSANTGNNERIINVSIKKLKRKPPSTNAGRRQKHRLTCPSCDSYEKKPPKEFLERFKSLLQKMIHQHLSSRTHGSEDSHHHHHH

SEQ ID NO: 60 - protein, 285 aa, synthetic construct
  REGION 1..285: note = hPD-1 D_hIL-21-6H
LDSPDRPWNPPTFSPALLVVTEGDNATFTCSFSNTSESFVLNWYRMSPSNQTDKLAAFPEDRSQPGQDCRFRVTQLPNGRDFHMSVVRARRNDSGTYLCGAISLAPKAQIKESLRAELRVTERRAEGGGGSGGGGSGGGGSHKSSSQGQDRHMIRMRQLIDIVDQLKNYVNDLVPEFLPAPEDVETNCEWSAFSCFQKAQLKSANTGNNERIINVSIKKLKRKPPSTNAGRRQKHRLTCPSCDSYEKKPPKEFLERFKSLLQKMIHQHLSSRTHGSEDSHHHHHH

SEQ ID NO: 61 - DNA, 930 bp, synthetic construct
  misc_feature 1..930: note = hPD-1 D_hIL-21-6H Polynucleotide
  source 1..930: mol_type = other DNA
atgcagatccctcaggctccatggccagtggtgtgggccgtgctccagctgggatggaggccaggctggttcctggactcccctgatcggccatggaatccccctacctttagcccagccctgctggtggtgacagagggcgacaacgctaccttcacatgctctttttccaacaccagcgagtctttcgtgctgaattggtacaggatgtcccccagcaaccagacagataagctggccgcttttccagaggaccggagccagcctggccaggattgcagattccgcgtgacccagctgcctaatggcagggactttcacatgtctgtggtgcgggccaggaggaacgattccggcacatacctgtgcggcgctatcagcctggccccaaaggctcagatcaaggagtccctgagagctgagctgagggtgaccgagagaagggctgagggaggaggaggctccggcggaggaggcagcggaggaggaggctctcacaagtccagctctcagggccaggatcgccacatgatcaggatgcggcagctgatcgacatcgtggatcagctgaagaactatgtgaatgacctggtgcctgagtttctgccagcccccgaggatgtggagaccaattgcgagtggtccgctttcagctgttttcagaaggcccagctgaagtctgctaatacaggcaacaatgagaggatcatcaacgtgagcatcaagaagctgaagcggaagcctccatctaccaacgctggcaggcggcagaagcacaggctgacatgcccttcttgtgactcctacgagaagaagccccctaaggagttcctggagaggttcaagtccctgctccagaagatgatccaccagcatctgtccagccgcacccatggcagcgaggattctcaccaccatcaccaccactga

SEQ ID NO: 62 - protein, 329 aa, synthetic construct
  REGION 1..329: note = hPD-1 ECD_hIL-21-6H with signal peptide
MQIPQAPWPVVWAVLQLGWRPGWFLDSPDRPWNPPTFSPALLVVTEGDNATFTCSFSNTSESFVLNWYRMSPSNQTDKLAAFPEDRSQPGQDCRFRVTQLPNGRDFHMSVVRARRNDSGTYLCGAISLAPKAQIKESLRAELRVTERRAEVPTAHPSPSPRPAGQFQTLVGGGGSGGGGSGGGGSHKSSSQGQDRHMIRMRQLIDIVDQLKNYVNDLVPEFLPAPEDVETNCEWSAFSCFQKAQLKSANTGNNERIINVSIKKLKRKPPSTNAGRRQKHRLTCPSCDSYEKKPPKEFLERFKSLLQKMIHQHLSSRTHGSEDSHHHHHH

SEQ ID NO: 63 - protein, 305 aa, synthetic construct
  REGION 1..305: note = hPD-1 ECD_hIL-21-6H
LDSPDRPWNPPTFSPALLVVTEGDNATFTCSFSNTSESFVLNWYRMSPSNQTDKLAAFPEDRSQPGQDCRFRVTQLPNGRDFHMSVVRARRNDSGTYLCGAISLAPKAQIKESLRAELRVTERRAEVPTAHPSPSPRPAGQFQTLVGGGGSGGGGSGGGGSHKSSSQGQDRHMIRMRQLIDIVDQLKNYVNDLVPEFLPAPEDVETNCEWSAFSCFQKAQLKSANTGNNERIINVSIKKLKRKPPSTNAGRRQKHRLTCPSCDSYEKKPPKEFLERFKSLLQKMIHQHLSSRTHGSEDSHHHHHH

SEQ ID NO: 64 - DNA, 990 bp, synthetic construct
  misc_feature 1..990: note = hPD-1 ECD_hIL-21-6H Polynucleotide
  source 1..990: mol_type = other DNA
atgcagatccctcaggctccatggccagtggtgtgggccgtgctccagctgggatggaggccaggctggttcctggactcccctgatcggccatggaatccccctacctttagcccagccctgctggtggtgacagagggcgacaacgctaccttcacatgctctttttccaacaccagcgagtctttcgtgctgaattggtacaggatgtcccccagcaaccagacagataagctggccgcttttccagaggaccggagccagcctggccaggattgcagattccgcgtgacccagctgcctaatggcagggactttcacatgtctgtggtgcgggccaggaggaacgattccggcacatacctgtgcggcgctatcagcctggccccaaaggctcagatcaaggagtccctgagagctgagctgagggtgaccgagagaagggctgaggttccaactgctcatccctctcctagcccccgccctgccggccaattccaaacactggtaggaggaggaggctccggcggaggaggcagcggaggaggaggctctcacaagtccagctctcagggccaggatcgccacatgatcaggatgcggcagctgatcgacatcgtggatcagctgaagaactatgtgaatgacctggtgcctgagtttctgccagcccccgaggatgtggagaccaattgcgagtggtccgctttcagctgttttcagaaggcccagctgaagtctgctaatacaggcaacaatgagaggatcatcaacgtgagcatcaagaagctgaagcggaagcctccatctaccaacgctggcaggcggcagaagcacaggctgacatgcccttcttgtgactcctacgagaagaagccccctaaggagttcctggagaggttcaagtccctgctccagaagatgatccaccagcatctgtccagccgcacccatggcagcgaggattctcaccaccatcaccaccactga

SEQ ID NO: 65 - protein, 304 aa, synthetic construct
  REGION 1..304: note = hIL-21_hPD-1 D-6H with signal peptide
MPRGWAAPLLLLLLQGGWGHKSSSQGQDRHMIRMRQLIDIVDQLKNYVNDLVPEFLPAPEDVETNCEWSAFSCFQKAQLKSANTGNNERIINVSIKKLKRKPPSTNAGRRQKHRLTCPSCDSYEKKPPKEFLERFKSLLQKMIHQHLSSRTHGSEDSGGGGSGGGGSGGGGSLDSPDRPWNPPTFSPALLVVTEGDNATFTCSFSNTSESFVLNWYRMSPSNQTDKLAAFPEDRSQPGQDCRFRVTQLPNGRDFHMSVVRARRNDSGTYLCGAISLAPKAQIKESLRAELRVTERRAEHHHHHH

SEQ ID NO: 66 - protein, 285 aa, synthetic construct
  REGION 1..285: note = hIL-21_hPD-1 D-6H
HKSSSQGQDRHMIRMRQLIDIVDQLKNYVNDLVPEFLPAPEDVETNCEWSAFSCFQKAQLKSANTGNNERIINVSIKKLKRKPPSTNAGRRQKHRLTCPSCDSYEKKPPKEFLERFKSLLQKMIHQHLSSRTHGSEDSGGGGSGGGGSGGGGSLDSPDRPWNPPTFSPALLVVTEGDNATFTCSFSNTSESFVLNWYRMSPSNQTDKLAAFPEDRSQPGQDCRFRVTQLPNGRDFHMSVVRARRNDSGTYLCGAISLAPKAQIKESLRAELRVTERRAEHHHHHH

SEQ ID NO: 67 - DNA, 915 bp, synthetic construct
  misc_feature 1..915: note = hIL-21_hPD-1 D-6H Polynucleotide
  source 1..915: mol_type = other DNA
atgccacgcggctgggctgctccactgctgctgctgctgctccagggcggctggggccacaagtccagctctcagggccaggatcgccacatgatcaggatgcggcagctgatcgacatcgtggatcagctgaagaactatgtgaatgacctggtgcctgagtttctgccagcccccgaggatgtggagaccaattgcgagtggtccgctttcagctgttttcagaaggcccagctgaagtctgctaatacaggcaacaatgagaggatcatcaacgtgagcatcaagaagctgaagcggaagcctccatctaccaacgctggcaggcggcagaagcacaggctgacatgcccttcttgtgactcctacgagaagaagccccctaaggagttcctggagaggttcaagtccctgctccagaagatgatccaccagcatctgtccagccgcacccatggcagcgaggattctggaggaggaggctccggcggaggaggcagcggaggaggaggctctctggactcccctgatcggccatggaatccccctacctttagcccagccctgctggtggtgacagagggcgacaacgctaccttcacatgctctttttccaacaccagcgagtctttcgtgctgaattggtacaggatgtcccccagcaaccagacagataagctggccgcttttccagaggaccggagccagcctggccaggattgcagattccgcgtgacccagctgcctaatggcagggactttcacatgtctgtggtgcgggccaggaggaacgattccggcacatacctgtgcggcgctatcagcctggccccaaaggctcagatcaaggagtccctgagagctgagctgagggtgaccgagagaagggctgagcaccaccatcaccaccactga

SEQ ID NO: 68 - protein, 324 aa, synthetic construct
  REGION 1..324: note = hIL-21_hPD-1 ECD-6H with signal peptide
MPRGWAAPLLLLLLQGGWGHKSSSQGQDRHMIRMRQLIDIVDQLKNYVNDLVPEFLPAPEDVETNCEWSAFSCFQKAQLKSANTGNNERIINVSIKKLKRKPPSTNAGRRQKHRLTCPSCDSYEKKPPKEFLERFKSLLQKMIHQHLSSRTHGSEDSGGGGSGGGGSGGGGSLDSPDRPWNPPTFSPALLVVTEGDNATFTCSFSNTSESFVLNWYRMSPSNQTDKLAAFPEDRSQPGQDCRFRVTQLPNGRDFHMSVVRARRNDSGTYLCGAISLAPKAQIKESLRAELRVTERRAEVPTAHPSPSPRPAGQFQTLVHHHHHH

SEQ ID NO: 69 - protein, 305 aa, synthetic construct
  REGION 1..305: note = hIL-21_hPD-1 ECD-6H
HKSSSQGQDRHMIRMRQLIDIVDQLKNYVNDLVPEFLPAPEDVETNCEWSAFSCFQKAQLKSANTGNNERIINVSIKKLKRKPPSTNAGRRQKHRLTCPSCDSYEKKPPKEFLERFKSLLQKMIHQHLSSRTHGSEDSGGGGSGGGGSGGGGSLDSPDRPWNPPTFSPALLVVTEGDNATFTCSFSNTSESFVLNWYRMSPSNQTDKLAAFPEDRSQPGQDCRFRVTQLPNGRDFHMSVVRARRNDSGTYLCGAISLAPKAQIKESLRAELRVTERRAEVPTAHPSPSPRPAGQFQTLVHHHHHH

SEQ ID NO: 70 - DNA, 975 bp, synthetic construct
  misc_feature 1..975: note = hIL-21_hPD-1 ECD-6H Polynucleotide
  source 1..975: mol_type = other DNA
atgccacgcggctgggctgctccactgctgctgctgctgctccagggcggctggggccacaagtccagctctcagggccaggatcgccacatgatcaggatgcggcagctgatcgacatcgtggatcagctgaagaactatgtgaatgacctggtgcctgagtttctgccagcccccgaggatgtggagaccaattgcgagtggtccgctttcagctgttttcagaaggcccagctgaagtctgctaatacaggcaacaatgagaggatcatcaacgtgagcatcaagaagctgaagcggaagcctccatctaccaacgctggcaggcggcagaagcacaggctgacatgcccttcttgtgactcctacgagaagaagccccctaaggagttcctggagaggttcaagtccctgctccagaagatgatccaccagcatctgtccagccgcacccatggcagcgaggattctggaggaggaggctccggcggaggaggcagcggaggaggaggctctctggactcccctgatcggccatggaatccccctacctttagcccagccctgctggtggtgacagagggcgacaacgctaccttcacatgctctttttccaacaccagcgagtctttcgtgctgaattggtacaggatgtcccccagcaaccagacagataagctggccgcttttccagaggaccggagccagcctggccaggattgcagattccgcgtgacccagctgcctaatggcagggactttcacatgtctgtggtgcgggccaggaggaacgattccggcacatacctgtgcggcgctatcagcctggccccaaaggctcagatcaaggagtccctgagagctgagctgagggtgaccgagagaagggctgaggttccaactgctcatccctctcctagcccccgccctgccggccaattccaaacactggtacaccaccatcaccaccactga

SEQ ID NO: 71 - protein, 217 aa, synthetic construct
  REGION 1..217: note = Fc(wt)_K
APELLGGPSVFLFPPKPKDTLMISRTPEVTCVVVDVSHEDPEVKFNWYVDGVEVHNAKTKPREEQYNSTYRVVSVLTVLHQDWLNGKEYKCKVSNKALPAPIEKTISKAKGQPREPQVYTLPPSRDELTKNQVSLTCLVKGFYPSDIAVEWESNGQPENNYKTTPPVLDSDGSFFLYSKLTVDKSRWQQGNVFSCSVMHEALHNHYTQKSLSLSPGK

SEQ ID NO: 72 - protein, 387 aa, synthetic construct
  REGION 1..387: note = hPD-1 D-Fc(wt) with signal peptide
MQIPQAPWPVVWAVLQLGWRPGWFLDSPDRPWNPPTFSPALLVVTEGDNATFTCSFSNTSESFVLNWYRMSPSNQTDKLAAFPEDRSQPGQDCRFRVTQLPNGRDFHMSVVRARRNDSGTYLCGAISLAPKAQIKESLRAELRVTERRAEGGGGSGGGGSDKTHTCPPCPAPELLGGPSVFLFPPKPKDTLMISRTPEVTCVVVDVSHEDPEVKFNWYVDGVEVHNAKTKPREEQYNSTYRVVSVLTVLHQDWLNGKEYKCKVSNKALPAPIEKTISKAKGQPREPQVYTLPPSRDELTKNQVSLTCLVKGFYPSDIAVEWESNGQPENNYKTTPPVLDSDGSFFLYSKLTVDKSRWQQGNVFSCSVMHEALHNHYTQKSLSLSPGK

SEQ ID NO: 73 - protein, 363 aa, synthetic construct
  REGION 1..363: note = hPD-1 D-Fc(wt)
LDSPDRPWNPPTFSPALLVVTEGDNATFTCSFSNTSESFVLNWYRMSPSNQTDKLAAFPEDRSQPGQDCRFRVTQLPNGRDFHMSVVRARRNDSGTYLCGAISLAPKAQIKESLRAELRVTERRAEGGGGSGGGGSDKTHTCPPCPAPELLGGPSVFLFPPKPKDTLMISRTPEVTCVVVDVSHEDPEVKFNWYVDGVEVHNAKTKPREEQYNSTYRVVSVLTVLHQDWLNGKEYKCKVSNKALPAPIEKTISKAKGQPREPQVYTLPPSRDELTKNQVSLTCLVKGFYPSDIAVEWESNGQPENNYKTTPPVLDSDGSFFLYSKLTVDKSRWQQGNVFSCSVMHEALHNHYTQKSLSLSPGK

SEQ ID NO: 74 - DNA, 1164 bp, synthetic construct
  misc_feature 1..1164: note = hPD-1 D-Fc(wt) Polynucleotide
  source 1..1164: mol_type = other DNA
atgcagatccctcaggctccatggccagtggtgtgggccgtgctccagctgggatggaggccaggctggttcctggactcccctgatcggccatggaatccccctacctttagcccagccctgctggtggtgacagagggcgacaacgctaccttcacatgctctttttccaacaccagcgagtctttcgtgctgaattggtacaggatgtcccccagcaaccagacagataagctggccgcttttccagaggaccggagccagcctggccaggattgcagattccgcgtgacccagctgcctaatggcagggactttcacatgtctgtggtgcgggccaggaggaacgattccggcacatacctgtgcggcgctatcagcctggccccaaaggctcagatcaaggagtccctgagagctgagctgagggtgaccgagagaagggctgagggaggaggaggctccggcggaggaggcagcgacaagacccatacatgcccaccatgtcctgctccagagctgctgggcggacctagcgtgttcctgtttcctccaaagccaaaggataccctgatgatctctaggaccccagaggtgacatgcgtggtggtggacgtgtcccacgaggaccccgaggtgaagttcaattggtacgtggacggcgtggaggtgcataacgctaagacaaagcccagagaggagcagtacaactctacctatcgcgtggtgtccgtgctgacagtgctgcaccaggattggctgaatggcaaggagtataagtgcaaggtgagcaacaaggccctgcccgctcctatcgagaagaccatctctaaggccaagggccagcccagagagcctcaggtgtacacactgcccccttccagggacgagctgaccaagaatcaggtgtccctgacatgtctggtgaagggcttctatccctccgacatcgctgtggagtgggagagcaacggccagcctgagaacaattacaagaccacaccacccgtgctggacagcgatggctctttctttctgtatagcaagctgaccgtggacaagtccaggtggcagcagggcaacgtgttctcctgctccgtgatgcatgaggccctgcacaaccattacacacagaagagcctgtctctgtcccccggcaagtga

SEQ ID NO: 75 - protein, 549 aa, synthetic construct
  REGION 1..549: note = hPD-1 ECD-Fc(wt)_hIL-21 with signal peptide
MQIPQAPWPVVWAVLQLGWRPGWFLDSPDRPWNPPTFSPALLVVTEGDNATFTCSFSNTSESFVLNWYRMSPSNQTDKLAAFPEDRSQPGQDCRFRVTQLPNGRDFHMSVVRARRNDSGTYLCGAISLAPKAQIKESLRAELRVTERRAEVPTAHPSPSPRPAGQFQTLVGGGGSGGGGSDKTHTCPPCPAPELLGGPSVFLFPPKPKDTLMISRTPEVTCVVVDVSHEDPEVKFNWYVDGVEVHNAKTKPREEQYNSTYRVVSVLTVLHQDWLNGKEYKCKVSNKALPAPIEKTISKAKGQPREPQVYTLPPSRDELTKNQVSLTCLVKGFYPSDIAVEWESNGQPENNYKTTPPVLDSDGSFFLYSKLTVDKSRWQQGNVFSCSVMHEALHNHYTQKSLSLSPGGGGGSHKSSSQGQDRHMIRMRQLIDIVDQLKNYVNDLVPEFLPAPEDVETNCEWSAFSCFQKAQLKSANTGNNERIINVSIKKLKRKPPSTNAGRRQKHRLTCPSCDSYEKKPPKEFLERFKSLLQKMIHQHLSSRTHGSEDS

SEQ ID NO: 76 - protein, 525 aa, synthetic construct
  REGION 1..525: note = hPD-1 ECD-Fc(wt)_hIL-21
LDSPDRPWNPPTFSPALLVVTEGDNATFTCSFSNTSESFVLNWYRMSPSNQTDKLAAFPEDRSQPGQDCRFRVTQLPNGRDFHMSVVRARRNDSGTYLCGAISLAPKAQIKESLRAELRVTERRAEVPTAHPSPSPRPAGQFQTLVGGGGSGGGGSDKTHTCPPCPAPELLGGPSVFLFPPKPKDTLMISRTPEVTCVVVDVSHEDPEVKFNWYVDGVEVHNAKTKPREEQYNSTYRVVSVLTVLHQDWLNGKEYKCKVSNKALPAPIEKTISKAKGQPREPQVYTLPPSRDELTKNQVSLTCLVKGFYPSDIAVEWESNGQPENNYKTTPPVLDSDGSFFLYSKLTVDKSRWQQGNVFSCSVMHEALHNHYTQKSLSLSPGGGGGSHKSSSQGQDRHMIRMRQLIDIVDQLKNYVNDLVPEFLPAPEDVETNCEWSAFSCFQKAQLKSANTGNNERIINVSIKKLKRKPPSTNAGRRQKHRLTCPSCDSYEKKPPKEFLERFKSLLQKMIHQHLSSRTHGSEDS

SEQ ID NO: 77 - DNA, 1650 bp, synthetic construct
  misc_feature 1..1650: note = hPD-1 ECD-Fc(wt)_hIL-21 Polynucleotide
  source 1..1650: mol_type = other DNA
atgcagatccctcaggctccatggccagtggtgtgggccgtgctccagctgggatggaggccaggctggttcctggactcccctgatcggccatggaatccccctacctttagcccagccctgctggtggtgacagagggcgacaacgctaccttcacatgctctttttccaacaccagcgagtctttcgtgctgaattggtacaggatgtcccccagcaaccagacagataagctggccgcttttccagaggaccggagccagcctggccaggattgcagattccgcgtgacccagctgcctaatggcagggactttcacatgtctgtggtgcgggccaggaggaacgattccggcacatacctgtgcggcgctatcagcctggccccaaaggctcagatcaaggagtccctgagagctgagctgagggtgaccgagagaagggctgaggttccaactgctcatccctctcctagcccccgccctgccggccaattccaaacactggtaggaggaggaggctccggcggaggaggcagcgacaagacccatacatgcccaccatgtcctgctccagagctgctgggcggacctagcgtgttcctgtttcctccaaagccaaaggataccctgatgatctctaggaccccagaggtgacatgcgtggtggtggacgtgtcccacgaggaccccgaggtgaagttcaattggtacgtggacggcgtggaggtgcataacgctaagacaaagcccagagaggagcagtacaactctacctatcgcgtggtgtccgtgctgacagtgctgcaccaggattggctgaatggcaaggagtataagtgcaaggtgagcaacaaggccctgcccgctcctatcgagaagaccatctctaaggccaagggccagcccagagagcctcaggtgtacacactgcccccttccagggacgagctgaccaagaatcaggtgtccctgacatgtctggtgaagggcttctatccctccgacatcgctgtggagtgggagagcaacggccagcctgagaacaattacaagaccacaccacccgtgctggacagcgatggctctttctttctgtatagcaagctgaccgtggacaagtccaggtggcagcagggcaacgtgttctcctgctccgtgatgcatgaggccctgcacaaccattacacacagaagagcctgtctctgtcccccggcggaggaggaggctctcacaagtccagctctcagggccaggatcgccacatgatcaggatgcggcagctgatcgacattgtggatcagctgaagaactatgtgaatgacctggtgcctgagtttctgccagcccccgaggatgtggagaccaattgcgagtggtccgctttcagctgttttcagaaggcccagctgaagtctgctaatacaggcaacaatgagaggatcatcaacgtgagcatcaagaagctgaagcggaagcctccatctaccaacgctggcaggcggcagaagcacagactgacatgcccttcttgtgactcctacgagaagaagccccctaaggagttcctggagaggttcaagtccctgctccagaagatgatccaccagcatctgtccagccgcacccatggcagcgaggattcttga

SEQ ID NO: 78 - protein, 534 aa, synthetic construct
  REGION 1..534: note = hIL-21_Fc(wt)_hPD-1 D with signal peptide
MPRGWAAPLLLLLLQGGWGHKSSSQGQDRHMIRMRQLIDIVDQLKNYVNDLVPEFLPAPEDVETNCEWSAFSCFQKAQLKSANTGNNERIINVSIKKLKRKPPSTNAGRRQKHRLTCPSCDSYEKKPPKEFLERFKSLLQKMIHQHLSSRTHGSEDSGGGGSDKTHTCPPCPAPELLGGPSVFLFPPKPKDTLMISRTPEVTCVVVDVSHEDPEVKFNWYVDGVEVHNAKTKPREEQYNSTYRVVSVLTVLHQDWLNGKEYKCKVSNKALPAPIEKTISKAKGQPREPQVYTLPPSRDELTKNQVSLTCLVKGFYPSDIAVEWESNGQPENNYKTTPPVLDSDGSFFLYSKLTVDKSRWQQGNVFSCSVMHEALHNHYTQKSLSLSPGGGGGSGGGGSGGGGSGGGGSLDSPDRPWNPPTFSPALLVVTEGDNATFTCSFSNTSESFVLNWYRMSPSNQTDKLAAFPEDRSQPGQDCRFRVTQLPNGRDFHMSVVRARRNDSGTYLCGAISLAPKAQIKESLRAELRVTERRAE

SEQ ID NO: 79 - protein, 515 aa, synthetic construct
  REGION 1..515: note = hIL-21_Fc(wt)_hPD-1 D
HKSSSQGQDRHMIRMRQLIDIVDQLKNYVNDLVPEFLPAPEDVETNCEWSAFSCFQKAQLKSANTGNNERIINVSIKKLKRKPPSTNAGRRQKHRLTCPSCDSYEKKPPKEFLERFKSLLQKMIHQHLSSRTHGSEDSGGGGSDKTHTCPPCPAPELLGGPSVFLFPPKPKDTLMISRTPEVTCVVVDVSHEDPEVKFNWYVDGVEVHNAKTKPREEQYNSTYRVVSVLTVLHQDWLNGKEYKCKVSNKALPAPIEKTISKAKGQPREPQVYTLPPSRDELTKNQVSLTCLVKGFYPSDIAVEWESNGQPENNYKTTPPVLDSDGSFFLYSKLTVDKSRWQQGNVFSCSVMHEALHNHYTQKSLSLSPGGGGGSGGGGSGGGGSGGGGSLDSPDRPWNPPTFSPALLVVTEGDNATFTCSFSNTSESFVLNWYRMSPSNQTDKLAAFPEDRSQPGQDCRFRVTQLPNGRDFHMSVVRARRNDSGTYLCGAISLAPKAQIKESLRAELRVTERRAE

SEQ ID NO: 80 - DNA, 1605 bp, synthetic construct
  misc_feature 1..1605: note = hIL-21_Fc(wt)_hPD-1 D Polynucleotide
  source 1..1605: mol_type = other DNA
atgccacgcggctgggctgctccactgctgctgctgctgctccagggcggctggggccacaagtccagctctcagggccaggatcgccacatgatcaggatgcggcagctgatcgacattgtggatcagctgaagaactatgtgaatgacctggtgcctgagtttctgccagcccccgaggatgtggagaccaattgcgagtggtccgctttcagctgttttcagaaggcccagctgaagtctgctaatacaggcaacaatgagaggatcatcaacgtgagcatcaagaagctgaagcggaagcctccatctaccaacgctggcaggcggcagaagcacagactgacatgcccttcttgtgactcctacgagaagaagccccctaaggagttcctggagaggttcaagtccctgctccagaagatgatccaccagcatctgtccagccgcacccatggcagcgaggattctggcggaggaggcagcgacaagacccatacatgcccaccatgtcctgctccagagctgctgggcggacctagcgtgttcctgtttcctccaaagccaaaggataccctgatgatctctaggaccccagaggtgacatgcgtggtggtggacgtgtcccacgaggaccccgaggtgaagttcaattggtacgtggacggcgtggaggtgcataacgctaagacaaagcccagagaggagcagtacaactctacctatcgcgtggtgtccgtgctgacagtgctgcaccaggattggctgaatggcaaggagtataagtgcaaggtgagcaacaaggccctgcccgctcctatcgagaagaccatctctaaggccaagggccagcccagagagcctcaggtgtacacactgcccccttccagggacgagctgaccaagaatcaggtgtccctgacatgtctggtgaagggcttctatccctccgacatcgctgtggagtgggagagcaacggccagcctgagaacaattacaagaccacaccacccgtgctggacagcgatggctctttctttctgtatagcaagctgaccgtggacaagtccaggtggcagcagggcaacgtgttctcctgctccgtgatgcatgaggccctgcacaaccattacacacagaagagcctgtctctgtcccccggcggaggaggaggctctggaggcggaggatccggaggtgggggaagcggtggtggtggcagcctggactcccctgatcggccatggaatccccctacctttagcccagccctgctggtggtgacagagggcgacaacgctaccttcacatgctctttttccaacaccagcgagtctttcgtgctgaattggtacaggatgtcccccagcaaccagacagataagctggccgcttttccagaggaccggagccagcctggccaggattgcagattccgcgtgacccagctgcctaatggcagggactttcacatgtctgtggtgcgggccaggaggaacgattccggcacatacctgtgcggcgctatcagcctggccccaaaggctcagatcaaggagtccctgagagctgagctgagggtgaccgagagaagggctgagtga

SEQ ID NO: 81 - protein, 554 aa, synthetic construct
  REGION 1..554: note = hIL-21_Fc(wt)_hPD-1 ECD with signal peptide
MPRGWAAPLLLLLLQGGWGHKSSSQGQDRHMIRMRQLIDIVDQLKNYVNDLVPEFLPAPEDVETNCEWSAFSCFQKAQLKSANTGNNERIINVSIKKLKRKPPSTNAGRRQKHRLTCPSCDSYEKKPPKEFLERFKSLLQKMIHQHLSSRTHGSEDSGGGGSDKTHTCPPCPAPELLGGPSVFLFPPKPKDTLMISRTPEVTCVVVDVSHEDPEVKFNWYVDGVEVHNAKTKPREEQYNSTYRVVSVLTVLHQDWLNGKEYKCKVSNKALPAPIEKTISKAKGQPREPQVYTLPPSRDELTKNQVSLTCLVKGFYPSDIAVEWESNGQPENNYKTTPPVLDSDGSFFLYSKLTVDKSRWQQGNVFSCSVMHEALHNHYTQKSLSLSPGGGGGSGGGGSGGGGSGGGGSLDSPDRPWNPPTFSPALLVVTEGDNATFTCSFSNTSESFVLNWYRMSPSNQTDKLAAFPEDRSQPGQDCRFRVTQLPNGRDFHMSVVRARRNDSGTYLCGAISLAPKAQIKESLRAELRVTERRAEVPTAHPSPSPRPAGQFQTLV

SEQ ID NO: 82 - protein, 535 aa, synthetic construct
  REGION 1..535: note = hIL-21_Fc(wt)_hPD-1 ECD
HKSSSQGQDRHMIRMRQLIDIVDQLKNYVNDLVPEFLPAPEDVETNCEWSAFSCFQKAQLKSANTGNNERIINVSIKKLKRKPPSTNAGRRQKHRLTCPSCDSYEKKPPKEFLERFKSLLQKMIHQHLSSRTHGSEDSGGGGSDKTHTCPPCPAPELLGGPSVFLFPPKPKDTLMISRTPEVTCVVVDVSHEDPEVKFNWYVDGVEVHNAKTKPREEQYNSTYRVVSVLTVLHQDWLNGKEYKCKVSNKALPAPIEKTISKAKGQPREPQVYTLPPSRDELTKNQVSLTCLVKGFYPSDIAVEWESNGQPENNYKTTPPVLDSDGSFFLYSKLTVDKSRWQQGNVFSCSVMHEALHNHYTQKSLSLSPGGGGGSGGGGSGGGGSGGGGSLDSPDRPWNPPTFSPALLVVTEGDNATFTCSFSNTSESFVLNWYRMSPSNQTDKLAAFPEDRSQPGQDCRFRVTQLPNGRDFHMSVVRARRNDSGTYLCGAISLAPKAQIKESLRAELRVTERRAEVPTAHPSPSPRPAGQFQTLV

SEQ ID NO: 83 - DNA, 1665 bp, synthetic construct
  misc_feature 1..1665: note = hIL-21_Fc(wt)_hPD-1 ECD Polynucleotide
  source 1..1665: mol_type = other DNA
atgccacgcggctgggctgctccactgctgctgctgctgctccagggcggctggggccacaagtccagctctcagggccaggatcgccacatgatcaggatgcggcagctgatcgacattgtggatcagctgaagaactatgtgaatgacctggtgcctgagtttctgccagcccccgaggatgtggagaccaattgcgagtggtccgctttcagctgttttcagaaggcccagctgaagtctgctaatacaggcaacaatgagaggatcatcaacgtgagcatcaagaagctgaagcggaagcctccatctaccaacgctggcaggcggcagaagcacagactgacatgcccttcttgtgactcctacgagaagaagccccctaaggagttcctggagaggttcaagtccctgctccagaagatgatccaccagcatctgtccagccgcacccatggcagcgaggattctggcggaggaggcagcgacaagacccatacatgcccaccatgtcctgctccagagctgctgggcggacctagcgtgttcctgtttcctccaaagccaaaggataccctgatgatctctaggaccccagaggtgacatgcgtggtggtggacgtgtcccacgaggaccccgaggtgaagttcaattggtacgtggacggcgtggaggtgcataacgctaagacaaagcccagagaggagcagtacaactctacctatcgcgtggtgtccgtgctgacagtgctgcaccaggattggctgaatggcaaggagtataagtgcaaggtgagcaacaaggccctgcccgctcctatcgagaagaccatctctaaggccaagggccagcccagagagcctcaggtgtacacactgcccccttccagggacgagctgaccaagaatcaggtgtccctgacatgtctggtgaagggcttctatccctccgacatcgctgtggagtgggagagcaacggccagcctgagaacaattacaagaccacaccacccgtgctggacagcgatggctctttctttctgtatagcaagctgaccgtggacaagtccaggtggcagcagggcaacgtgttctcctgctccgtgatgcatgaggccctgcacaaccattacacacagaagagcctgtctctgtcccccggcggaggaggaggctctggaggcggaggatccggaggtgggggaagcggtggtggtggcagcctggactcccctgatcggccatggaatccccctacctttagcccagccctgctggtggtgacagagggcgacaacgctaccttcacatgctctttttccaacaccagcgagtctttcgtgctgaattggtacaggatgtcccccagcaaccagacagataagctggccgcttttccagaggaccggagccagcctggccaggattgcagattccgcgtgacccagctgcctaatggcagggactttcacatgtctgtggtgcgggccaggaggaacgattccggcacatacctgtgcggcgctatcagcctggccccaaaggctcagatcaaggagtccctgagagctgagctgagggtgaccgagagaagggctgaggttccaactgctcatccctctcctagcccccgccctgccggccaattccaaacactggtatga

SEQ ID NO: 84 - protein, 388 aa, synthetic construct
  REGION 1..388: note = Fc(wt)_hIL-21 with signal peptide
MPRGWAAPLLLLLLQGGWGDKTHTCPPCPAPELLGGPSVFLFPPKPKDTLMISRTPEVTCVVVDVSHEDPEVKFNWYVDGVEVHNAKTKPREEQYNSTYRVVSVLTVLHQDWLNGKEYKCKVSNKALPAPIEKTISKAKGQPREPQVYTLPPSRDELTKNQVSLTCLVKGFYPSDIAVEWESNGQPENNYKTTPPVLDSDGSFFLYSKLTVDKSRWQQGNVFSCSVMHEALHNHYTQKSLSLSPGGGGGSHKSSSQGQDRHMIRMRQLIDIVDQLKNYVNDLVPEFLPAPEDVETNCEWSAFSCFQKAQLKSANTGNNERIINVSIKKLKRKPPSTNAGRRQKHRLTCPSCDSYEKKPPKEFLERFKSLLQKMIHQHLSSRTHGSEDS

SEQ ID NO: 85 - protein, 369 aa, synthetic construct
  REGION 1..369: note = Fc(wt)_hIL-21
DKTHTCPPCPAPELLGGPSVFLFPPKPKDTLMISRTPEVTCVVVDVSHEDPEVKFNWYVDGVEVHNAKTKPREEQYNSTYRVVSVLTVLHQDWLNGKEYKCKVSNKALPAPIEKTISKAKGQPREPQVYTLPPSRDELTKNQVSLTCLVKGFYPSDIAVEWESNGQPENNYKTTPPVLDSDGSFFLYSKLTVDKSRWQQGNVFSCSVMHEALHNHYTQKSLSLSPGGGGGSHKSSSQGQDRHMIRMRQLIDIVDQLKNYVNDLVPEFLPAPEDVETNCEWSAFSCFQKAQLKSANTGNNERIINVSIKKLKRKPPSTNAGRRQKHRLTCPSCDSYEKKPPKEFLERFKSLLQKMIHQHLSSRTHGSEDS

SEQ ID NO: 86 - DNA, 1167 bp, synthetic construct
  misc_feature 1..1167: note = Fc(wt)_hIL-21 Polynucleotide
  source 1..1167: mol_type = other DNA
atgccacgcggctgggctgctccactgctgctgctgctgctccagggcggctggggcgacaagacccatacatgcccaccatgtcctgctccagagctgctgggcggacctagcgtgttcctgtttcctccaaagccaaaggataccctgatgatctctaggaccccagaggtgacatgcgtggtggtggacgtgtcccacgaggaccccgaggtgaagttcaattggtacgtggacggcgtggaggtgcataacgctaagacaaagcccagagaggagcagtacaactctacctatcgcgtggtgtccgtgctgacagtgctgcaccaggattggctgaatggcaaggagtataagtgcaaggtgagcaacaaggccctgcccgctcctatcgagaagaccatctctaaggccaagggccagcccagagagcctcaggtgtacacactgcccccttccagggacgagctgaccaagaatcaggtgtccctgacatgtctggtgaagggcttctatccctccgacatcgctgtggagtgggagagcaacggccagcctgagaacaattacaagaccacaccacccgtgctggacagcgatggctctttctttctgtatagcaagctgaccgtggacaagtccaggtggcagcagggcaacgtgttctcctgctccgtgatgcatgaggccctgcacaaccattacacacagaagagcctgtctctgtcccccggcggaggaggaggctctcacaagtccagctctcagggccaggatcgccacatgatcaggatgcggcagctgatcgacattgtggatcagctgaagaactatgtgaatgacctggtgcctgagtttctgccagcccccgaggatgtggagaccaattgcgagtggtccgctttcagctgttttcagaaggcccagctgaagtctgctaatacaggcaacaatgagaggatcatcaacgtgagcatcaagaagctgaagcggaagcctccatctaccaacgctggcaggcggcagaagcacagactgacatgcccttcttgtgactcctacgagaagaagccccctaaggagttcctggagaggttcaagtccctgctccagaagatgatccaccagcatctgtccagccgcacccatggcagcgaggattcttga

SEQ ID NO: 87 - protein, 216 aa, synthetic construct
  REGION 1..216: note = Fc(wt, K)
APELLGGPSVFLFPPKPKDTLMISRTPEVTCVVVDVSHEDPEVKFNWYVDGVEVHNAKTKPREEQYNSTYRVVSVLTVLHQDWLNGKEYKCKVSNKALPAPIEKTISKAKGQPREPQVYTLPPSRDELTKNQVSLWCLVKGFYPSDIAVEWESNGQPENNYKTTPPVLDSDGSFFLYSKLTVDKSRWQQGNVFSCSVMHEALHNHYTQKSLSLSPG

SEQ ID NO: 88 - protein, 529 aa, synthetic construct
  REGION 1..529: note = hPD-1 D-Fc(wt, K)_hIL-21 with signal peptide
MQIPQAPWPVVWAVLQLGWRPGWFLDSPDRPWNPPTFSPALLVVTEGDNATFTCSFSNTSESFVLNWYRMSPSNQTDKLAAFPEDRSQPGQDCRFRVTQLPNGRDFHMSVVRARRNDSGTYLCGAISLAPKAQIKESLRAELRVTERRAEGGGGSGGGGSDKTHTCPPCPAPELLGGPSVFLFPPKPKDTLMISRTPEVTCVVVDVSHEDPEVKFNWYVDGVEVHNAKTKPREEQYNSTYRVVSVLTVLHQDWLNGKEYKCKVSNKALPAPIEKTISKAKGQPREPQVYTLPPSRDELTKNQVSLWCLVKGFYPSDIAVEWESNGQPENNYKTTPPVLDSDGSFFLYSKLTVDKSRWQQGNVFSCSVMHEALHNHYTQKSLSLSPGGGGGSHKSSSQGQDRHMIRMRQLIDIVDQLKNYVNDLVPEFLPAPEDVETNCEWSAFSCFQKAQLKSANTGNNERIINVSIKKLKRKPPSTNAGRRQKHRLTCPSCDSYEKKPPKEFLERFKSLLQKMIHQHLSSRTHGSEDS

SEQ ID NO: 89 - protein, 505 aa, synthetic construct
  REGION 1..505: note = hPD-1 D-Fc(wt, K)_hIL-21
LDSPDRPWNPPTFSPALLVVTEGDNATFTCSFSNTSESFVLNWYRMSPSNQTDKLAAFPEDRSQPGQDCRFRVTQLPNGRDFHMSVVRARRNDSGTYLCGAISLAPKAQIKESLRAELRVTERRAEGGGGSGGGGSDKTHTCPPCPAPELLGGPSVFLFPPKPKDTLMISRTPEVTCVVVDVSHEDPEVKFNWYVDGVEVHNAKTKPREEQYNSTYRVVSVLTVLHQDWLNGKEYKCKVSNKALPAPIEKTISKAKGQPREPQVYTLPPSRDELTKNQVSLWCLVKGFYPSDIAVEWESNGQPENNYKTTPPVLDSDGSFFLYSKLTVDKSRWQQGNVFSCSVMHEALHNHYTQKSLSLSPGGGGGSHKSSSQGQDRHMIRMRQLIDIVDQLKNYVNDLVPEFLPAPEDVETNCEWSAFSCFQKAQLKSANTGNNERIINVSIKKLKRKPPSTNAGRRQKHRLTCPSCDSYEKKPPKEFLERFKSLLQKMIHQHLSSRTHGSEDS

SEQ ID NO: 90 - DNA, 1590 bp, synthetic construct
  misc_feature 1..1590: note = hPD-1 D-Fc(wt, K)_hIL-21 Polynucleotide
  source 1..1590: mol_type = other DNA
atgcagatccctcaggctccatggccagtggtgtgggccgtgctccagctgggatggaggccaggctggttcctggactcccctgatcggccatggaatccccctacctttagcccagccctgctggtggtgacagagggcgacaacgctaccttcacatgctctttttccaacaccagcgagtctttcgtgctgaattggtacaggatgtcccccagcaaccagacagataagctggccgcttttccagaggaccggagccagcctggccaggattgcagattccgcgtgacccagctgcctaatggcagggactttcacatgtctgtggtgcgggccaggaggaacgattccggcacatacctgtgcggcgctatcagcctggccccaaaggctcagatcaaggagtccctgagagctgagctgagggtgaccgagagaagggctgagggaggaggaggctccggcggaggaggcagcgacaagacccatacatgcccaccatgtcctgctccagagctgctgggcggacctagcgtgttcctgtttcctccaaagccaaaggataccctgatgatctctaggaccccagaggtgacatgcgtggtggtggacgtgtcccacgaggaccccgaggtgaagttcaattggtacgtggacggcgtggaggtgcataacgctaagacaaagcccagagaggagcagtacaactctacctatcgcgtggtgtccgtgctgacagtgctgcaccaggattggctgaatggcaaggagtataagtgcaaggtgagcaacaaggccctgcccgctcctatcgagaagaccatctctaaggccaagggccagcccagagagcctcaggtgtacacactgcccccttccagggacgagctgaccaagaatcaggtgtccctgtggtgtctggtgaagggcttctatccctccgacatcgctgtggagtgggagagcaacggccagcctgagaacaattacaagaccacaccacccgtgctggacagcgatggctctttctttctgtatagcaagctgaccgtggacaagtccaggtggcagcagggcaacgtgttctcctgctccgtgatgcatgaggccctgcacaaccattacacacagaagagcctgtctctgtcccccggcggaggaggaggctctcacaagtccagctctcagggccaggatcgccacatgatcaggatgcggcagctgatcgacattgtggatcagctgaagaactatgtgaatgacctggtgcctgagtttctgccagcccccgaggatgtggagaccaattgcgagtggtccgctttcagctgttttcagaaggcccagctgaagtctgctaatacaggcaacaatgagaggatcatcaacgtgagcatcaagaagctgaagcggaagcctccatctaccaacgctggcaggcggcagaagcacagactgacatgcccttcttgtgactcctacgagaagaagccccctaaggagttcctggagaggttcaagtccctgctccagaagatgatccaccagcatctgtccagccgcacccatggcagcgaggattcttga

SEQ ID NO: 91 - protein, 520 aa, synthetic construct
  REGION 1..520: note = hPD-1 D-Fc(wt, K)_mIL-21 with signal peptide
MQIPQAPWPVVWAVLQLGWRPGWFLDSPDRPWNPPTFSPALLVVTEGDNATFTCSFSNTSESFVLNWYRMSPSNQTDKLAAFPEDRSQPGQDCRFRVTQLPNGRDFHMSVVRARRNDSGTYLCGAISLAPKAQIKESLRAELRVTERRAEGGGGSGGGGSDKTHTCPPCPAPELLGGPSVFLFPPKPKDTLMISRTPEVTCVVVDVSHEDPEVKFNWYVDGVEVHNAKTKPREEQYNSTYRVVSVLTVLHQDWLNGKEYKCKVSNKALPAPIEKTISKAKGQPREPQVYTLPPSRDELTKNQVSLWCLVKGFYPSDIAVEWESNGQPENNYKTTPPVLDSDGSFFLYSKLTVDKSRWQQGNVFSCSVMHEALHNHYTQKSLSLSPGGGGGSHKSSPQGPDRLLIRLRHLIDIVEQLKIYENDLDPELLSAPQDVKGHCEHAAFACFQKAKLKPSNPGNNKTFIIDLVAQLRRRLPARRGGKKQKHIAKCPSCDSYEKRTPKEFLERLKWLLQKMIHQHLS

SEQ ID NO: 92 - protein, 496 aa, synthetic construct
  REGION 1..496: note = hPD-1 D-Fc(wt, K)_mIL-21
LDSPDRPWNPPTFSPALLVVTEGDNATFTCSFSNTSESFVLNWYRMSPSNQTDKLAAFPEDRSQPGQDCRFRVTQLPNGRDFHMSVVRARRNDSGTYLCGAISLAPKAQIKESLRAELRVTERRAEGGGGSGGGGSDKTHTCPPCPAPELLGGPSVFLFPPKPKDTLMISRTPEVTCVVVDVSHEDPEVKFNWYVDGVEVHNAKTKPREEQYNSTYRVVSVLTVLHQDWLNGKEYKCKVSNKALPAPIEKTISKAKGQPREPQVYTLPPSRDELTKNQVSLWCLVKGFYPSDIAVEWESNGQPENNYKTTPPVLDSDGSFFLYSKLTVDKSRWQQGNVFSCSVMHEALHNHYTQKSLSLSPGGGGGSHKSSPQGPDRLLIRLRHLIDIVEQLKIYENDLDPELLSAPQDVKGHCEHAAFACFQKAKLKPSNPGNNKTFIIDLVAQLRRRLPARRGGKKQKHIAKCPSCDSYEKRTPKEFLERLKWLLQKMIHQHLS

SEQ ID NO: 93 - DNA, 1563 bp, synthetic construct
  misc_feature 1..1563: note = hPD-1 D-Fc(wt, K)_mIL-21 Polynucleotide
  source 1..1563: mol_type = other DNA
atgcagatccctcaggctccatggccagtggtgtgggccgtgctccagctgggatggaggccaggctggttcctggactcccctgatcggccatggaatccccctacctttagcccagccctgctggtggtgacagagggcgacaacgctaccttcacatgctctttttccaacaccagcgagtctttcgtgctgaattggtacaggatgtcccccagcaaccagacagataagctggccgcttttccagaggaccggagccagcctggccaggattgcagattccgcgtgacccagctgcctaatggcagggactttcacatgtctgtggtgcgggccaggaggaacgattccggcacatacctgtgcggcgctatcagcctggccccaaaggctcagatcaaggagtccctgagagctgagctgagggtgaccgagagaagggctgagggaggaggaggctccggcggaggaggcagcgacaagacccatacatgcccaccatgtcctgctccagagctgctgggcggacctagcgtgttcctgtttcctccaaagccaaaggataccctgatgatctctaggaccccagaggtgacatgcgtggtggtggacgtgtcccacgaggaccccgaggtgaagttcaattggtacgtggacggcgtggaggtgcataacgctaagacaaagcccagagaggagcagtacaactctacctatcgcgtggtgtccgtgctgacagtgctgcaccaggattggctgaatggcaaggagtataagtgcaaggtgagcaacaaggccctgcccgctcctatcgagaagaccatctctaaggccaagggccagcccagagagcctcaggtgtacacactgcccccttccagggacgagctgaccaagaatcaggtgtccctgtggtgtctggtgaagggcttctatccctccgacatcgctgtggagtgggagagcaacggccagcctgagaacaattacaagaccacaccacccgtgctggacagcgatggctctttctttctgtatagcaagctgaccgtggacaagtccaggtggcagcagggcaacgtgttctcctgctccgtgatgcatgaggccctgcacaaccattacacacagaagagcctgtctctgtcccccggcggaggaggaggctctcataagagtagcccccaaggtccagacagactgcttatccgacttagacatctcatagacatcgttgagcaacttaaaatctatgaaaatgacctggaccctgagctgctgtctgctccacaggatgtaaagggtcactgcgaacatgctgctttcgcttgttttcagaaggcaaaactgaaaccatcaaatcccggcaataataagactttcattatagacctggttgctcaactgcgtcgaaggctccctgcacgacgaggtggtaagaaacaaaaacacatcgctaaatgccccagttgtgattcctatgagaagcgcacccctaaggagttcttggaaaggctcaagtggcttctccagaaaatgatccatcagcatctctcatga

SEQ ID NO: 94 - protein, 19 aa, synthetic construct
  REGION 1..19: note = Signal Peptide 3
MEWSWVFLFFLSVTTGVHS

SEQ ID NO: 95 - protein, 215 aa, synthetic construct
  REGION 1..215: note = Fc(29)R
APPVAGPSVFLFPPKPKDTLMISRTPEVTCVVVDVSHEDPEVKFNWYVDGVEVHNAKTKPREEQYNSTYRVVSVLTVLHRDWLNGKEYKCKVSNKALPAPIEKTISKAKGQPREPQVYTLPPSRDELTKNQVSLTCLVKGFYPSDIAVEWESNGQPENNYKTTPPVLDSDGSFFLYSKLTVDKSRWQQGNVFSCSVLHEALHNHYTQKSLSLSPG

SEQ ID NO: 96 - protein, 523 aa, synthetic construct
  REGION 1..523: note = hPD-1 D-Fc(29)R-hIL-21 with signal peptide
MEWSWVFLFFLSVTTGVHSLDSPDRPWNPPTFSPALLVVTEGDNATFTCSFSNTSESFVLNWYRMSPSNQTDKLAAFPEDRSQPGQDCRFRVTQLPNGRDFHMSVVRARRNDSGTYLCGAISLAPKAQIKESLRAELRVTERRAEGGGGSGGGGSDKTHTCPPCPAPPVAGPSVFLFPPKPKDTLMISRTPEVTCVVVDVSHEDPEVKFNWYVDGVEVHNAKTKPREEQYNSTYRVVSVLTVLHRDWLNGKEYKCKVSNKALPAPIEKTISKAKGQPREPQVYTLPPSRDELTKNQVSLTCLVKGFYPSDIAVEWESNGQPENNYKTTPPVLDSDGSFFLYSKLTVDKSRWQQGNVFSCSVLHEALHNHYTQKSLSLSPGGGGGSHKSSSQGQDRHMIRMRQLIDIVDQLKNYVNDLVPEFLPAPEDVETNCEWSAFSCFQKAQLKSANTGNNERIINVSIKKLKRKPPSTNAGRRQKHRLTCPSCDSYEKKPPKEFLERFKSLLQKMIHQHLSSRTHGSEDS

SEQ ID NO: 97 - protein, 504 aa, synthetic construct
  REGION 1..504: note = hPD-1 D-Fc(29)R-hIL-21
LDSPDRPWNPPTFSPALLVVTEGDNATFTCSFSNTSESFVLNWYRMSPSNQTDKLAAFPEDRSQPGQDCRFRVTQLPNGRDFHMSVVRARRNDSGTYLCGAISLAPKAQIKESLRAELRVTERRAEGGGGSGGGGSDKTHTCPPCPAPPVAGPSVFLFPPKPKDTLMISRTPEVTCVVVDVSHEDPEVKFNWYVDGVEVHNAKTKPREEQYNSTYRVVSVLTVLHRDWLNGKEYKCKVSNKALPAPIEKTISKAKGQPREPQVYTLPPSRDELTKNQVSLTCLVKGFYPSDIAVEWESNGQPENNYKTTPPVLDSDGSFFLYSKLTVDKSRWQQGNVFSCSVLHEALHNHYTQKSLSLSPGGGGGSHKSSSQGQDRHMIRMRQLIDIVDQLKNYVNDLVPEFLPAPEDVETNCEWSAFSCFQKAQLKSANTGNNERIINVSIKKLKRKPPSTNAGRRQKHRLTCPSCDSYEKKPPKEFLERFKSLLQKMIHQHLSSRTHGSEDS

SEQ ID NO: 98 - DNA, 1572 bp, synthetic construct
  misc_feature 1..1572: note = hPD-1 D-Fc(29)R-hIL-21 Polynucleotide
  source 1..1572: mol_type = other DNA
atggagtggtcctgggtgttcctcttcttcctgtccgtgactactggggtgcactccctggattcgcctgatcgcccctggaaccctccgaccttttcccctgcgctcctggtcgtgaccgagggcgataacgccaccttcacctgttcattctccaacaccagcgagagcttcgtgctcaactggtacaggatgagcccaagcaaccagaccgacaagctcgccgcgtttcccgaggatcgatcacagccggggcaggattgccggttccgcgtgactcagctgcccaatggccgcgacttccacatgagcgtcgtcagagcacggcggaatgactccggaacctacttgtgcggggccattagcctggcacctaaggcccagatcaaggagtccctgagagctgaactgcgcgtgaccgaacggagagctgagggtggcggaggctctggtggaggagggtccgacaagactcacacttgcccaccgtgtcctgcaccgcccgtggccggtccgtcggtgttcttgttcccgcccaaacccaaggacaccctgatgatctcacggactcctgaggtcacctgtgtggtcgtggatgtgtcccatgaggacccggaagtcaagttcaattggtacgtggacggagtggaggtgcacaacgccaagacaaagccccgggaggaacagtacaattccacctatcgcgtcgtgtccgtgctcaccgtgctgcaccgggactggcttaacggaaaggagtacaagtgcaaagtgtccaacaaggccttgcctgctccgattgaaaagactatcagcaaggccaaagggcagcccagggaaccccaagtgtacaccctgccaccgtcgagggacgagctgaccaagaaccaagtgtcccttacttgcctcgtgaagggattctacccgtccgacatcgccgtggagtgggaatccaacggacagcccgagaacaactacaagactacgcctcccgtgctggacagcgacggctcgttcttcctgtattcgaagctcaccgtggacaagtcccgctggcaacagggcaacgtgttctcatgctcggtgctccatgaagccctgcacaaccactacacccagaaatccctgagcctgagcccaggaggaggaggcggatcacacaaatcgtcctcgcaagggcaggatagacacatgatcagaatgagacaactgatcgacatcgtcgatcagctgaagaattacgtgaacgatctggtgccggagttcctgccagccccagaggacgtcgaaaccaactgcgaatggagcgcgttcagctgcttccagaaagcccaacttaagtccgccaacaccggcaacaacgagaggatcatcaacgtgtccatcaagaagctgaagaggaaaccgccttccaccaacgccggcaggagacagaagcaccgcctgacttgcccgtcctgcgatagctacgaaaagaagcctccgaaggaattcctggaacgctttaagtcactgctgcaaaagatgatccatcagcacctgagttcccggactcacggcagcgaagattcgtaa

SEQ ID NO: 99 - protein, 215 aa, synthetic construct
  REGION 1..215: note = Fc(29)RE
APPVAGPDVFLFPPKPKDTLMISRTPEVTCVVVDVSHEDPEVKFNWYVDGVEVHNAKTKPREEQYNSTYRVVSVLTVLHRDWLNGKEYKCKVSNKALPAPEEKTISKAKGQPREPQVYTLPPSRDELTKNQVSLTCLVKGFYPSDIAVEWESNGQPENNYKTTPPVLDSDGSFFLYSKLTVDKSRWQQGNVFSCSVLHEALHNHYTQKSLSLSPG

SEQ ID NO: 100 - protein, 523 aa, synthetic construct
  REGION 1..523: note = hPD-1 D-Fc(29)RE-hIL-21 with signal peptide
MEWSWVFLFFLSVTTGVHSLDSPDRPWNPPTFSPALLVVTEGDNATFTCSFSNTSESFVLNWYRMSPSNQTDKLAAFPEDRSQPGQDCRFRVTQLPNGRDFHMSVVRARRNDSGTYLCGAISLAPKAQIKESLRAELRVTERRAEGGGGSGGGGSDKTHTCPPCPAPPVAGPDVFLFPPKPKDTLMISRTPEVTCVVVDVSHEDPEVKFNWYVDGVEVHNAKTKPREEQYNSTYRVVSVLTVLHRDWLNGKEYKCKVSNKALPAPEEKTISKAKGQPREPQVYTLPPSRDELTKNQVSLTCLVKGFYPSDIAVEWESNGQPENNYKTTPPVLDSDGSFFLYSKLTVDKSRWQQGNVFSCSVLHEALHNHYTQKSLSLSPGGGGGSHKSSSQGQDRHMIRMRQLIDIVDQLKNYVNDLVPEFLPAPEDVETNCEWSAFSCFQKAQLKSANTGNNERIINVSIKKLKRKPPSTNAGRRQKHRLTCPSCDSYEKKPPKEFLERFKSLLQKMIHQHLSSRTHGSEDS

SEQ ID NO: 101 - protein, 504 aa, synthetic construct
  REGION 1..504: note = hPD-1 D-Fc(29)RE-hIL-21
LDSPDRPWNPPTFSPALLVVTEGDNATFTCSFSNTSESFVLNWYRMSPSNQTDKLAAFPEDRSQPGQDCRFRVTQLPNGRDFHMSVVRARRNDSGTYLCGAISLAPKAQIKESLRAELRVTERRAEGGGGSGGGGSDKTHTCPPCPAPPVAGPDVFLFPPKPKDTLMISRTPEVTCVVVDVSHEDPEVKFNWYVDGVEVHNAKTKPREEQYNSTYRVVSVLTVLHRDWLNGKEYKCKVSNKALPAPEEKTISKAKGQPREPQVYTLPPSRDELTKNQVSLTCLVKGFYPSDIAVEWESNGQPENNYKTTPPVLDSDGSFFLYSKLTVDKSRWQQGNVFSCSVLHEALHNHYTQKSLSLSPGGGGGSHKSSSQGQDRHMIRMRQLIDIVDQLKNYVNDLVPEFLPAPEDVETNCEWSAFSCFQKAQLKSANTGNNERIINVSIKKLKRKPPSTNAGRRQKHRLTCPSCDSYEKKPPKEFLERFKSLLQKMIHQHLSSRTHGSEDS

SEQ ID NO: 102 - protein, 1572 aa, synthetic construct
  REGION 1..1572: note = hPD-1 D-Fc(29)RE-hIL-21 Polynucleotide
ATGGAGTGGTCCTGGGTGTTCCTCTTCTTCCTGTCCGTGACTACTGGGGTGCACTCCCTGGATTCGCCTGATCGCCCCTGGAACCCTCCGACCTTTTCCCCTGCGCTCCTGGTCGTGACCGAGGGCGATAACGCCACCTTCACCTGTTCATTCTCCAACACCAGCGAGAGCTTCGTGCTCAACTGGTACAGGATGAGCCCAAGCAACCAGACCGACAAGCTCGCCGCGTTTCCCGAGGATCGATCACAGCCGGGGCAGGATTGCCGGTTCCGCGTGACTCAGCTGCCCAATGGCCGCGACTTCCACATGAGCGTCGTCAGAGCACGGCGGAATGACTCCGGAACCTACTTGTGCGGGGCCATTAGCCTGGCACCTAAGGCCCAGATCAAGGAGTCCCTGAGAGCTGAACTGCGCGTGACCGAACGGAGAGCTGAGGGTGGCGGAGGCTCTGGTGGAGGAGGGTCCGACAAGACTCACACTTGCCCACCGTGTCCTGCACCGCCCGTGGCCGGTCCGGACGTGTTCTTGTTCCCGCCCAAACCCAAGGACACCCTGATGATCTCACGGACTCCTGAGGTCACCTGTGTGGTCGTGGATGTGTCCCATGAGGACCCGGAAGTCAAGTTCAATTGGTACGTGGACGGAGTGGAGGTGCACAACGCCAAGACAAAGCCCCGGGAGGAACAGTACAATTCCACCTATCGCGTCGTGTCCGTGCTCACCGTGCTGCACCGGGACTGGCTTAACGGAAAGGAGTACAAGTGCAAAGTGTCCAACAAGGCCTTGCCTGCTCCGGAGGAAAAGACTATCAGCAAGGCCAAAGGGCAGCCCAGGGAACCCCAAGTGTACACCCTGCCACCGTCGAGGGACGAGCTGACCAAGAACCAAGTGTCCCTTACTTGCCTCGTGAAGGGATTCTACCCGTCCGACATCGCCGTGGAGTGGGAATCCAACGGACAGCCCGAGAACAACTACAAGACTACGCCTCCCGTGCTGGACAGCGACGGCTCGTTCTTCCTGTATTCGAAGCTCACCGTGGACAAGTCCCGCTGGCAACAGGGCAACGTGTTCTCATGCTCGGTGCTCCATGAAGCCCTGCACAACCACTACACCCAGAAATCCCTGAGCCTGAGCCCAGGAGGAGGAGGCGGATCACACAAATCGTCCTCGCAAGGGCAGGATAGACACATGATCAGAATGAGACAACTGATCGACATCGTCGATCAGCTGAAGAATTACGTGAACGATCTGGTGCCGGAGTTCCTGCCAGCCCCAGAGGACGTCGAAACCAACTGCGAATGGAGCGCGTTCAGCTGCTTCCAGAAAGCCCAACTTAAGTCCGCCAACACCGGCAACAACGAGAGGATCATCAACGTGTCCATCAAGAAGCTGAAGAGGAAACCGCCTTCCACCAACGCCGGCAGGAGACAGAAGCACCGCCTGACTTGCCCGTCCTGCGATAGCTACGAAAAGAAGCCTCCGAAGGAATTCCTGGAACGCTTTAAGTCACTGCTGCAAAAGATGATCCATCAGCACCTGAGTTCCCGGACTCACGGCAGCGAAGATTCGTAA

SEQ ID NO: 103 - protein, 126 aa, synthetic construct
  REGION 1..126: note = hPD-1v
LDSPDRPWNPPTFSPALLVVTEGDNATFTCSFSNTSESFVLNWYRMSPSNQTDKLAAFPEDRSQPGQDCRFRVTQLPNGRDFHMSVVRARRNDSGTYLCGAISLRPKAQIKESLRAELRVTERRAE

SEQ ID NO: 104 - protein, 215 aa, synthetic construct; identical to SEQ ID NO: 99
  REGION 1..215: note = Fc(29)REA

SEQ ID NO: 105 - protein, 523 aa, synthetic construct
  REGION 1..523: note = hPD-1v D-Fc(29)REA-hIL-21 with signal peptide
MEWSWVFLFFLSVTTGVHSLDSPDRPWNPPTFSPALLVVTEGDNATFTCSFSNTSESFVLNWYRMSPSNQTDKLAAFPEDRSQPGQDCRFRVTQLPNGRDFHMSVVRARRNDSGTYLCGAISLRPKAQIKESLRAELRVTERRAEGGGGSGGGGSDKTHTCPPCPAPPVAGPDVFLFPPKPKDTLMISRTPEVTCVVVDVSHEDPEVKFNWYVDGVEVHNAKTKPREEQYNSTYRVVSVLTVLHRDWLNGKEYKCKVSNKALPAPEEKTISKAKGQPREPQVYTLPPSRDELTKNQVSLTCLVKGFYPSDIAVEWESNGQPENNYKTTPPVLDSDGSFFLYSKLTVDKSRWQQGNVFSCSVLHEALHNHYTQKSLSLSPGGGGGSHKSSSQGQDRHMIRMRQLIDIVDQLKNYVNDLVPEFLPAPEDVETNCEWSAFSCFQKAQLKSANTGNNERIINVSIKKLKRKPPSTNAGRRQKHRLTCPSCDSYEKKPPKEFLERFKSLLQKMIHQHLSSRTHGSEDS

SEQ ID NO: 106 - protein, 504 aa, synthetic construct
  REGION 1..504: note = hPD-1v D-Fc(29)REA-hIL-21
LDSPDRPWNPPTFSPALLVVTEGDNATFTCSFSNTSESFVLNWYRMSPSNQTDKLAAFPEDRSQPGQDCRFRVTQLPNGRDFHMSVVRARRNDSGTYLCGAISLRPKAQIKESLRAELRVTERRAEGGGGSGGGGSDKTHTCPPCPAPPVAGPDVFLFPPKPKDTLMISRTPEVTCVVVDVSHEDPEVKFNWYVDGVEVHNAKTKPREEQYNSTYRVVSVLTVLHRDWLNGKEYKCKVSNKALPAPEEKTISKAKGQPREPQVYTLPPSRDELTKNQVSLTCLVKGFYPSDIAVEWESNGQPENNYKTTPPVLDSDGSFFLYSKLTVDKSRWQQGNVFSCSVLHEALHNHYTQKSLSLSPGGGGGSHKSSSQGQDRHMIRMRQLIDIVDQLKNYVNDLVPEFLPAPEDVETNCEWSAFSCFQKAQLKSANTGNNERIINVSIKKLKRKPPSTNAGRRQKHRLTCPSCDSYEKKPPKEFLERFKSLLQKMIHQHLSSRTHGSEDS

SEQ ID NO: 107 - DNA, 1572 bp, synthetic construct
  misc_feature 1..1572: note = hPD-1v D-Fc(29)REA-hIL-21 Polynucleotide
  source 1..1572: mol_type = other DNA
atggagtggtcctgggtgttcctcttcttcctgtccgtgactactggggtgcactccctggattcgcctgatcgcccctggaaccctccgaccttttcccctgcgctcctggtcgtgaccgagggcgataacgccaccttcacctgttcattctccaacaccagcgagagcttcgtgctcaactggtacaggatgagcccaagcaaccagaccgacaagctcgccgcgtttcccgaggatcgatcacagccggggcaggattgccggttccgcgtgactcagctgcccaatggccgcgacttccacatgagcgtcgtcagagcacggcggaatgactccggaacctacttgtgcggggccattagcctgaggcctaaggcccagatcaaggagtccctgagagctgaactgcgcgtgaccgaacggagagctgagggtggcggaggctctggtggaggagggtccgacaagactcacacttgcccaccgtgtcctgcaccgcccgtggccggtccggacgtgttcttgttcccgcccaaacccaaggacaccctgatgatctcacggactcctgaggtcacctgtgtggtcgtggatgtgtcccatgaggacccggaagtcaagttcaattggtacgtggacggagtggaggtgcacaacgccaagacaaagccccgggaggaacagtacaattccacctatcgcgtcgtgtccgtgctcaccgtgctgcaccgggactggcttaacggaaaggagtacaagtgcaaagtgtccaacaaggccttgcctgctccggaggaaaagactatcagcaaggccaaagggcagcccagggaaccccaagtgtacaccctgccaccgtcgagggacgagctgaccaagaaccaagtgtcccttacttgcctcgtgaagggattctacccgtccgacatcgccgtggagtgggaatccaacggacagcccgagaacaactacaagactacgcctcccgtgctggacagcgacggctcgttcttcctgtattcgaagctcaccgtggacaagtcccgctggcaacagggcaacgtgttctcatgctcggtgctccatgaagccctgcacaaccactacacccagaaatccctgagcctgagcccaggaggaggaggcggatcacacaaatcgtcctcgcaagggcaggatagacacatgatcagaatgagacaactgatcgacatcgtcgatcagctgaagaattacgtgaacgatctggtgccggagttcctgccagccccagaggacgtcgaaaccaactgcgaatggagcgcgttcagctgcttccagaaagcccaacttaagtccgccaacaccggcaacaacgagaggatcatcaacgtgtccatcaagaagctgaagaggaaaccgccttccaccaacgccggcaggagacagaagcaccgcctgacttgcccgtcctgcgatagctacgaaaagaagcctccgaaggaattcctggaacgctttaagtcactgctgcaaaagatgatccatcagcacctgagttcccggactcacggcagcgaagattcgtaa

SEQ ID NO: 108 - protein, 215 aa, synthetic construct
  REGION 1..215: note = Fc(wt)R
APPVAGPSVFLFPPKPKDTLMISRTPEVTCVVVDVSHEDPEVKFNWYVDGVEVHNAKTKPREEQYNSTYRVVSVLTVLHQDWLNGKEYKCKVSNKALPAPIEKTISKAKGQPREPQVYTLPPSRDELTKNQVSLTCLVKGFYPSDIAVEWESNGQPENNYKTTPPVLDSDGSFFLYSKLTVDKSRWQQGNVFSCSVMHEALHNHYTQKSLSLSPG

SEQ ID NO: 109 - protein, 523 aa, synthetic construct
  REGION 1..523: note = hPD-1 D-Fc(wt)R-hIL-21 with signal peptide
MEWSWVFLFFLSVTTGVHSLDSPDRPWNPPTFSPALLVVTEGDNATFTCSFSNTSESFVLNWYRMSPSNQTDKLAAFPEDRSQPGQDCRFRVTQLPNGRDFHMSVVRARRNDSGTYLCGAISLAPKAQIKESLRAELRVTERRAEGGGGSGGGGSDKTHTCPPCPAPPVAGPSVFLFPPKPKDTLMISRTPEVTCVVVDVSHEDPEVKFNWYVDGVEVHNAKTKPREEQYNSTYRVVSVLTVLHQDWLNGKEYKCKVSNKALPAPIEKTISKAKGQPREPQVYTLPPSRDELTKNQVSLTCLVKGFYPSDIAVEWESNGQPENNYKTTPPVLDSDGSFFLYSKLTVDKSRWQQGNVFSCSVMHEALHNHYTQKSLSLSPGGGGGSHKSSSQGQDRHMIRMRQLIDIVDQLKNYVNDLVPEFLPAPEDVETNCEWSAFSCFQKAQLKSANTGNNERIINVSIKKLKRKPPSTNAGRRQKHRLTCPSCDSYEKKPPKEFLERFKSLLQKMIHQHLSSRTHGSEDS

SEQ ID NO: 110 - protein, 504 aa, synthetic construct
  REGION 1..504: note = hPD-1 D-Fc(wt)R-hIL-21
LDSPDRPWNPPTFSPALLVVTEGDNATFTCSFSNTSESFVLNWYRMSPSNQTDKLAAFPEDRSQPGQDCRFRVTQLPNGRDFHMSVVRARRNDSGTYLCGAISLAPKAQIKESLRAELRVTERRAEGGGGSGGGGSDKTHTCPPCPAPPVAGPSVFLFPPKPKDTLMISRTPEVTCVVVDVSHEDPEVKFNWYVDGVEVHNAKTKPREEQYNSTYRVVSVLTVLHQDWLNGKEYKCKVSNKALPAPIEKTISKAKGQPREPQVYTLPPSRDELTKNQVSLTCLVKGFYPSDIAVEWESNGQPENNYKTTPPVLDSDGSFFLYSKLTVDKSRWQQGNVFSCSVMHEALHNHYTQKSLSLSPGGGGGSHKSSSQGQDRHMIRMRQLIDIVDQLKNYVNDLVPEFLPAPEDVETNCEWSAFSCFQKAQLKSANTGNNERIINVSIKKLKRKPPSTNAGRRQKHRLTCPSCDSYEKKPPKEFLERFKSLLQKMIHQHLSSRTHGSEDS

SEQ ID NO: 111 - DNA, 1572 bp, synthetic construct
  misc_feature 1..1572: note = hPD-1 D-Fc(wt)R-hIL-21 Polynucleotide
  source 1..1572: mol_type = other DNA
atggagtggtcctgggtgttcctcttcttcctgtccgtgactactggggtgcactccctggattcgcctgatcgcccctggaaccctccgaccttttcccctgcgctcctggtcgtgaccgagggcgataacgccaccttcacctgttcattctccaacaccagcgagagcttcgtgctcaactggtacaggatgagcccaagcaaccagaccgacaagctcgccgcgtttcccgaggatcgatcacagccggggcaggattgccggttccgcgtgactcagctgcccaatggccgcgacttccacatgagcgtcgtcagagcacggcggaatgactccggaacctacttgtgcggggccattagcctggcacctaaggcccagatcaaggagtccctgagagctgaactgcgcgtgaccgaacggagagctgagggtggcggaggctctggtggaggagggtccgacaagactcacacttgcccaccgtgtcctgcaccgcccgtggccggtccgtcggtgttcttgttcccgcccaaacccaaggacaccctgatgatctcacggactcctgaggtcacctgtgtggtcgtggatgtgtcccatgaggacccggaagtcaagttcaattggtacgtggacggagtggaggtgcacaacgccaagacaaagccccgggaggaacagtacaattccacctatcgcgtcgtgtccgtgctcaccgtgctgcaccaggactggcttaacggaaaggagtacaagtgcaaagtgtccaacaaggccttgcctgctccgattgaaaagactatcagcaaggccaaagggcagcccagggaaccccaagtgtacaccctgccaccgtcgagggacgagctgaccaagaaccaagtgtcccttacttgcctcgtgaagggattctacccgtccgacatcgccgtggagtgggaatccaacggacagcccgagaacaactacaagactacgcctcccgtgctggacagcgacggctcgttcttcctgtattcgaagctcaccgtggacaagtcccgctggcaacagggcaacgtgttctcatgctcggtgatgcatgaagccctgcacaaccactacacccagaaatccctgagcctgagcccaggaggaggaggcggatcacacaaatcgtcctcgcaagggcaggatagacacatgatcagaatgagacaactgatcgacatcgtcgatcagctgaagaattacgtgaacgatctggtgccggagttcctgccagccccagaggacgtcgaaaccaactgcgaatggagcgcgttcagctgcttccagaaagcccaacttaagtccgccaacaccggcaacaacgagaggatcatcaacgtgtccatcaagaagctgaagaggaaaccgccttccaccaacgccggcaggagacagaagcaccgcctgacttgcccgtcctgcgatagctacgaaaagaagcctccgaaggaattcctggaacgctttaagtcactgctgcaaaagatgatccatcagcacctgagttcccggactcacggcagcgaagattcgtaa

SEQ ID NO: 112 - protein, 215 aa, synthetic construct
  REGION 1..215: note = Fc(wt)RE
APPVAGPDVFLFPPKPKDTLMISRTPEVTCVVVDVSHEDPEVKFNWYVDGVEVHNAKTKPREEQYNSTYRVVSVLTVLHQDWLNGKEYKCKVSNKALPAPEEKTISKAKGQPREPQVYTLPPSRDELTKNQVSLTCLVKGFYPSDIAVEWESNGQPENNYKTTPPVLDSDGSFFLYSKLTVDKSRWQQGNVFSCSVMHEALHNHYTQKSLSLSPG

SEQ ID NO: 113 - protein, 523 aa, synthetic construct
  REGION 1..523: note = hPD-1 D-Fc(wt)RE-hIL-21 with signal peptide
MEWSWVFLFFLSVTTGVHSLDSPDRPWNPPTFSPALLVVTEGDNATFTCSFSNTSESFVLNWYRMSPSNQTDKLAAFPEDRSQPGQDCRFRVTQLPNGRDFHMSVVRARRNDSGTYLCGAISLAPKAQIKESLRAELRVTERRAEGGGGSGGGGSDKTHTCPPCPAPPVAGPDVFLFPPKPKDTLMISRTPEVTCVVVDVSHEDPEVKFNWYVDGVEVHNAKTKPREEQYNSTYRVVSVLTVLHQDWLNGKEYKCKVSNKALPAPEEKTISKAKGQPREPQVYTLPPSRDELTKNQVSLTCLVKGFYPSDIAVEWESNGQPENNYKTTPPVLDSDGSFFLYSKLTVDKSRWQQGNVFSCSVMHEALHNHYTQKSLSLSPGGGGGSHKSSSQGQDRHMIRMRQLIDIVDQLKNYVNDLVPEFLPAPEDVETNCEWSAFSCFQKAQLKSANTGNNERIINVSIKKLKRKPPSTNAGRRQKHRLTCPSCDSYEKKPPKEFLERFKSLLQKMIHQHLSSRTHGSEDS

SEQ ID NO: 114 - protein, 504 aa, synthetic construct
  REGION 1..504: note = hPD-1 D-Fc(wt)RE-hIL-21
LDSPDRPWNPPTFSPALLVVTEGDNATFTCSFSNTSESFVLNWYRMSPSNQTDKLAAFPEDRSQPGQDCRFRVTQLPNGRDFHMSVVRARRNDSGTYLCGAISLAPKAQIKESLRAELRVTERRAEGGGGSGGGGSDKTHTCPPCPAPPVAGPDVFLFPPKPKDTLMISRTPEVTCVVVDVSHEDPEVKFNWYVDGVEVHNAKTKPREEQYNSTYRVVSVLTVLHQDWLNGKEYKCKVSNKALPAPEEKTISKAKGQPREPQVYTLPPSRDELTKNQVSLTCLVKGFYPSDIAVEWESNGQPENNYKTTPPVLDSDGSFFLYSKLTVDKSRWQQGNVFSCSVMHEALHNHYTQKSLSLSPGGGGGSHKSSSQGQDRHMIRMRQLIDIVDQLKNYVNDLVPEFLPAPEDVETNCEWSAFSCFQKAQLKSANTGNNERIINVSIKKLKRKPPSTNAGRRQKHRLTCPSCDSYEKKPPKEFLERFKSLLQKMIHQHLSSRTHGSEDS

SEQ ID NO: 115 - DNA, 1572 bp, synthetic construct
  misc_feature 1..1572: note = hPD-1 D-Fc(wt)RE-hIL-21 Polynucleotide
  source 1..1572: mol_type = other DNA
atggagtggtcctgggtgttcctcttcttcctgtccgtgactactggggtgcactccctggattcgcctgatcgcccctggaaccctccgaccttttcccctgcgctcctggtcgtgaccgagggcgataacgccaccttcacctgttcattctccaacaccagcgagagcttcgtgctcaactggtacaggatgagcccaagcaaccagaccgacaagctcgccgcgtttcccgaggatcgatcacagccggggcaggattgccggttccgcgtgactcagctgcccaatggccgcgacttccacatgagcgtcgtcagagcacggcggaatgactccggaacctacttgtgcggggccattagcctggcacctaaggcccagatcaaggagtccctgagagctgaactgcgcgtgaccgaacggagagctgagggtggcggaggctctggtggaggagggtccgacaagactcacacttgcccaccgtgtcctgcaccgcccgtggccggtccggacgtgttcttgttcccgcccaaacccaaggacaccctgatgatctcacggactcctgaggtcacctgtgtggtcgtggatgtgtcccatgaggacccggaagtcaagttcaattggtacgtggacggagtggaggtgcacaacgccaagacaaagccccgggaggaacagtacaattccacctatcgcgtcgtgtccgtgctcaccgtgctgcaccaggactggcttaacggaaaggagtacaagtgcaaagtgtccaacaaggccttgcctgctccggaggaaaagactatcagcaaggccaaagggcagcccagggaaccccaagtgtacaccctgccaccgtcgagggacgagctgaccaagaaccaagtgtcccttacttgcctcgtgaagggattctacccgtccgacatcgccgtggagtgggaatccaacggacagcccgagaacaactacaagactacgcctcccgtgctggacagcgacggctcgttcttcctgtattcgaagctcaccgtggacaagtcccgctggcaacagggcaacgtgttctcatgctcggtgatgcatgaagccctgcacaaccactacacccagaaatccctgagcctgagcccaggaggaggaggcggatcacacaaatcgtcctcgcaagggcaggatagacacatgatcagaatgagacaactgatcgacatcgtcgatcagctgaagaattacgtgaacgatctggtgccggagttcctgccagccccagaggacgtcgaaaccaactgcgaatggagcgcgttcagctgcttccagaaagcccaacttaagtccgccaacaccggcaacaacgagaggatcatcaacgtgtccatcaagaagctgaagaggaaaccgccttccaccaacgccggcaggagacagaagcaccgcctgacttgcccgtcctgcgatagctacgaaaagaagcctccgaaggaattcctggaacgctttaagtcactgctgcaaaagatgatccatcagcacctgagttcccggactcacggcagcgaagattcgtaa

SEQ ID NO: 116 - protein, 215 aa, synthetic construct; identical to SEQ ID NO: 112
  REGION 1..215: note = Fc(wt)REA

SEQ ID NO: 117 - protein, 523 aa, synthetic construct
  REGION 1..523: note = hPD-1v D-Fc(wt)REA-hIL-21 with signal peptide
MEWSWVFLFFLSVTTGVHSLDSPDRPWNPPTFSPALLVVTEGDNATFTCSFSNTSESFVLNWYRMSPSNQTDKLAAFPEDRSQPGQDCRFRVTQLPNGRDFHMSVVRARRNDSGTYLCGAISLRPKAQIKESLRAELRVTERRAEGGGGSGGGGSDKTHTCPPCPAPPVAGPDVFLFPPKPKDTLMISRTPEVTCVVVDVSHEDPEVKFNWYVDGVEVHNAKTKPREEQYNSTYRVVSVLTVLHQDWLNGKEYKCKVSNKALPAPEEKTISKAKGQPREPQVYTLPPSRDELTKNQVSLTCLVKGFYPSDIAVEWESNGQPENNYKTTPPVLDSDGSFFLYSKLTVDKSRWQQGNVFSCSVMHEALHNHYTQKSLSLSPGGGGGSHKSSSQGQDRHMIRMRQLIDIVDQLKNYVNDLVPEFLPAPEDVETNCEWSAFSCFQKAQLKSANTGNNERIINVSIKKLKRKPPSTNAGRRQKHRLTCPSCDSYEKKPPKEFLERFKSLLQKMIHQHLSSRTHGSEDS

SEQ ID NO: 118 - protein, 504 aa, synthetic construct
  REGION 1..504: note = hPD-1v D-Fc(wt)REA-hIL-21
LDSPDRPWNPPTFSPALLVVTEGDNATFTCSFSNTSESFVLNWYRMSPSNQTDKLAAFPEDRSQPGQDCRFRVTQLPNGRDFHMSVVRARRNDSGTYLCGAISLRPKAQIKESLRAELRVTERRAEGGGGSGGGGSDKTHTCPPCPAPPVAGPDVFLFPPKPKDTLMISRTPEVTCVVVDVSHEDPEVKFNWYVDGVEVHNAKTKPREEQYNSTYRVVSVLTVLHQDWLNGKEYKCKVSNKALPAPEEKTISKAKGQPREPQVYTLPPSRDELTKNQVSLTCLVKGFYPSDIAVEWESNGQPENNYKTTPPVLDSDGSFFLYSKLTVDKSRWQQGNVFSCSVMHEALHNHYTQKSLSLSPGGGGGSHKSSSQGQDRHMIRMRQLIDIVDQLKNYVNDLVPEFLPAPEDVETNCEWSAFSCFQKAQLKSANTGNNERIINVSIKKLKRKPPSTNAGRRQKHRLTCPSCDSYEKKPPKEFLERFKSLLQKMIHQHLSSRTHGSEDS

SEQ ID NO: 119 - DNA, 1572 bp, synthetic construct
  misc_feature 1..1572: note = hPD-1v D-Fc(wt)REA-hIL-21 Polynucleotide
  source 1..1572: mol_type = other DNA
atggagtggtcctgggtgttcctcttcttcctgtccgtgactactggggtgcactccctggattcgcctgatcgcccctggaaccctccgaccttttcccctgcgctcctggtcgtgaccgagggcgataacgccaccttcacctgttcattctccaacaccagcgagagcttcgtgctcaactggtacaggatgagcccaagcaaccagaccgacaagctcgccgcgtttcccgaggatcgatcacagccggggcaggattgccggttccgcgtgactcagctgcccaatggccgcgacttccacatgagcgtcgtcagagcacggcggaatgactccggaacctacttgtgcggggccattagcctgaggcctaaggcccagatcaaggagtccctgagagctgaactgcgcgtgaccgaacggagagctgagggtggcggaggctctggtggaggagggtccgacaagactcacacttgcccaccgtgtcctgcaccgcccgtggccggtccggacgtgttcttgttcccgcccaaacccaaggacaccctgatgatctcacggactcctgaggtcacctgtgtggtcgtggatgtgtcccatgaggacccggaagtcaagttcaattggtacgtggacggagtggaggtgcacaacgccaagacaaagccccgggaggaacagtacaattccacctatcgcgtcgtgtccgtgctcaccgtgctgcaccaggactggcttaacggaaaggagtacaagtgcaaagtgtccaacaaggccttgcctgctccggaggaaaagactatcagcaaggccaaagggcagcccagggaaccccaagtgtacaccctgccaccgtcgagggacgagctgaccaagaaccaagtgtcccttacttgcctcgtgaagggattctacccgtccgacatcgccgtggagtgggaatccaacggacagcccgagaacaactacaagactacgcctcccgtgctggacagcgacggctcgttcttcctgtattcgaagctcaccgtggacaagtcccgctggcaacagggcaacgtgttctcatgctcggtgatgcatgaagccctgcacaaccactacacccagaaatccctgagcctgagcccaggaggaggaggcggatcacacaaatcgtcctcgcaagggcaggatagacacatgatcagaatgagacaactgatcgacatcgtcgatcagctgaagaattacgtgaacgatctggtgccggagttcctgccagccccagaggacgtcgaaaccaactgcgaatggagcgcgttcagctgcttccagaaagcccaacttaagtccgccaacaccggcaacaacgagaggatcatcaacgtgtccatcaagaagctgaagaggaaaccgccttccaccaacgccggcaggagacagaagcaccgcctgacttgcccgtcctgcgatagctacgaaaagaagcctccgaaggaattcctggaacgctttaagtcactgctgcaaaagatgatccatcagcacctgagttcccggactcacggcagcgaagattcgtaa

SEQ ID NO: 120 - DNA, 21 bp, synthetic construct
  misc_feature 1..21: note = PD-L1-forward
  source 1..21: mol_type = other DNA
tggcatttgctgaacgcattt

SEQ ID NO: 121 - DNA, 22 bp, synthetic construct
  misc_feature 1..22: note = PD-L1-reverse
  source 1..22: mol_type = other DNA
tgcagccaggtctaattgtttt

SEQ ID NO: 122 - DNA, 20 bp, synthetic construct
  misc_feature 1..20: note = PD-L2-forward
  source 1..20: mol_type = other DNA
cagcaatgtgaccctggaat

SEQ ID NO: 123 - DNA, 21 bp, synthetic construct
  misc_feature 1..21: note = PD-L2-reverse
  source 1..21: mol_type = other DNA
ggacttgaggtatgtggaacg

SEQ ID NO: 124 - DNA, 20 bp, synthetic construct
  misc_feature 1..20: note = PD-1-forward
  source 1..20: mol_type = other DNA
tgcagcttctccaacacatc

SEQ ID NO: 125 - DNA, 20 bp, synthetic construct
  misc_feature 1..20: note = PD-1-reverse
  source 1..20: mol_type = other DNA
ctgcccttctctctgtcacc

SEQ ID NO: 126 - DNA, 20 bp, synthetic construct
  misc_feature 1..20: note = GAPDH-2-forward
  source 1..20: mol_type = other DNA
agccgcatcttcttttgcgt

SEQ ID NO: 127 - DNA, 20 bp, synthetic construct
  misc_feature 1..20: note = GAPDH-2-reverse
  source 1..20: mol_type = other DNA
tgacgaacatgggggcatca